European Patent Specification EP 3 568 483 B1, published August 13, 2025. Title: POLYNUCLEOTIDES AND VECTORS FOR THE EXPRESSION OF TRANSGENES. Applicant: Children's Medical Research Institute The Sydney Children's Hospitals Network (Randwick and Westmead) (incorporating the Royal Alexandra Hospital for Children). The sequence listing filed with the application follows.

SEQUENCE LISTING (36 sequences)

SEQ ID NO: 1 - DNA, 2232 bp, Homo sapiens
acaagaaagttaaaattgaattagaggaatcatggggtcaacaagagcccctggatgaattctgaggatgaacatcaaagcctgtaaagtaaaacagactccacatgtgacataatcagcagaagctgggtagttgaaatctacccctcaacaagttcattgagatgccctgccttttgagattcagtgaaattgcttttaacttcatcccacttgtgatgcagctccccttttccaatccctctgggagttattggtatcttaacttttttttagttccctctggctttgagctcctgcatctgtagcattaggagggtttgtgagttgctttggcatctcagaaatgctgcctgtactctctagcatggaactgcagacacttcttgatttctccccaagcattaccaatatgagttgtgtgtatggctagcacagttcagtgaagatatggggtcaagctatgggctttatattagcctgtggtttggcctcatctccctcaggctccatgcaaacgttcaatttcactcctgtattatgtggagcgcttttgctctctgaaacctattcaataactggccttgtttgcctcttcaaagatgctttattatgttttttaaattcactctctcccttctcacctctgtacctttgcaagcagttgcttctgcctggaatatcctttccagaatggaagatttggtagaggttgggaaatgtcagtctttcccctcactttatctcacatcattctctgtaagtagaaggaaatggtgacaatatttatttctctactagtattaattatgacatcacaaacatctcggctcctgaggtggccatagttggtctttaaataacactttttggtattccacaaacttctggaaaatatttacttgggtttgctaaagtcatataaattgaccagaagaggcagccctacccctgcccctcctctccttcctcctacccttcctaccttagagggctcccgcttcttcgaagccagacaactttgtctggacctctcctatgggcttgtattatggatatttgtttataaatcataccacctttactgaactgtgaactctgcaaagatgatgtcatcttccctctctgaaacttcagtgcagctcggtatctgatacagaattgactttgaatcacctgatttctaactgaggataaatgaataaatgtgaagttgcagatggccccttagtgatctgaataggctgctaggggaagagcatatggtatccccacttcccacttgtactgactgtcaggtgctgttagaatcaataggcaactatttcttttctttttctttctttctttcttttttttgagacagtgtctctctctgtcacccaggctggagtacagtggtgcaatctgggctcactgcaacctctgtctcccgggttcaagcgactctcatgcctcagcctcccaaatagctgggattacaggtgtgcaccaccacgtctagctaatttttgtatttttagtggagacggggattcaccatgttggccaggctggtctcgaactcctgggctcaagtgatccgcccgcctcagcctcccaaagtgctgggattacaggcgtgagccaccgtgcccggccagcaattatttctttattgaagacttatgtgcaaggcacaaagggagctccaggactgagatatttttactataccttctctatcatcttgcacccccaaaatagcttccagggcacttctttctatttgtttttgtggaaagactggcaattagaggtagaaaagtgaaataaatggaaatagtactactcaggactgtcacatctacatctgtgtttttgcagtgccaatttgcattttctgagtgagttacttctactcaccttcacagcagccggtaccgcagtgccttgcatatattatatcctcaatgagtacttgtcaattgattttgtacatgcgtgtgacagtataaatatattatgaaaaatgaggaggccaggcaataaaagagtcaggatttcttccaaaaaaaatacacagcggtggagcttggcataaagttcaaatgctcctacaccctgccctgcagtatctctaaccaggggactttgataaggaagctgaagggtgatattacctttgctccctcactgcaactgaacacatttcttagtttttaggtggcccccgctggctaacttgctgtg

SEQ ID NO: 2 - DNA, 789 bp, Homo sapiens
caagcgactctcatgcctcagcctcccaaatagctgggattacaggtgtgcaccaccacgtctagctaatttttgtatttttagtggagacggggattcatcatgttggccaggctggtctcgaactcctgggctcaagtgatccgcccgcctcagcctcccaaagtgctgggattataggcgtgagccaccatgcccggccagcaattatttctttattgaagacttatgtgcaaggcacaaagggagctccaggactgagatatttttactataccttctctatcatcttgcacccccaaaatagcttccagggcacttctatttgtttttgtggaaagactggcaattagaggtagaaaagtgaaataaatggaaatagtactactcagggctgtcacatctacatctgtgtttttgcagtgccaatttgcattttctgagtgagttacttctactcaccttcacagcagccagtaccgcagtgccttgcatatattatatcctcaatgagtacttgtcaattgattttgtacatgcgtgtgacagtataaatatattatgaaaaatgaggaggccaggcaataaaagagtcaggatttcttccaaaaaaaatacacagcggtggagcttggcataaagttcaaatgctcctacaccctgccctgcagtatctctaaccaggggactttgataaggaagctgaagggtgatattacctttgctccctcactgcaactgaacacatttcttagtttttaggtggcccccgctggctaacttgctgtg

SEQ ID NO: 3 - DNA, 2232 bp, Homo sapiens
cccagtcttgtgtctgccgggcaatgagcaaggctccttcctgtccaagctccccgcccctccccagcctactgcctccacccgaagtctacttcctgggtgggcaggaactgggcactgtgcccagggcatgcactgcctccacgcagcaaccctcagagtcctgagctgaaccaagaaggaggagggggtcgggcctccgaggaaggcctagccgctgctgctgccaggaattccaggttggaggggcggcaacctcctgccagccttcaggccactctcctgtgcctgccagaagagacagagcttgaggagagcttgaggagagcaggaaaggtgggacattgctgctgctgctcactcagttccacaggtgggagggacagcagggcttagagtgggggtcattgtgcagatgggaaaacaaaggcccagagaggggaagaaatgcccaggagctaccgagggcaggcgacctcaaccacagcccagtgctggagctgtgagtggatgtagagcagcggaatatccattcagccagctcaggggaaggacaggggccctgaagccaggggatggagctgcagggaagggagctcagagagaaggggaggggagtctgagctcagtttcccgctgcctgaaaggagggtggtacctactcccttcacagggtaactgaatgagagactgcctggaggaaagctcttcaagtgtggcccaccccaccccagtgacaccagcccctgacacgggggagggagggcagcatcaggaggggctttctgggcacacccagtacccgtctctgagctttccttgaactgttgcattttaatcctcacagcagctcaacaaggtacataccgtcaccatccccattttacagatagggaaattgaggctcggagcggttaaacaactcacctgaggcctcacagccagtaagtgggttccctggtctgaatgtgtgtgctggaggatcctgtgggtcactcgcctggtagagccccaaggtggaggcataaatgggactggtgaatgacagaaggggcaaaaatgcactcatccattcactctgcaagtatctacggcacgtacgccagctcccaagcaggtttgcgggttgcacagcgggcgatgcaatctgatttaggcttttaaagggattgcaatcaagtggggccccactagcctcaaccctgtacctcccctcccctccacccccagcagtctccaaaggcctccaacaaccccagagtgggggccatgtatccaaagaaactccaagctgtatacggatcacactggttttccaggagcaaaaacagaaacaggcctgaggctggtcaaaattgaacctcctcctgctctgagcagcctggggggcagactaagcagagggctgtgcagacccacataaagagcctactgtgtgccaggcacttcacccgaggcacttcacaagcatgcttgggaatgaaacttccaactctttgggatgcaggtgaaacagttcctggttcagagaggtgaagcggcctgcctgaggcagcacagctcttctttacagatgtgcttccccacctctaccctgtctcacggccccccatgccagcctgacggttgtgtctgcctcagtcatgctccatttttccatcgggaccatcaagagggtgtttgtgtctaaggctgactgggtaactttggatgagcggtctctccgctctgagcctgtttcctcatctgtcaaatgggctctaacccactctgatctcccagggcggcagtaagtcttcagcatcaggcattttggggtgactcagtaaatggtagatcttgctaccagtggaacagccactaaggattctgcagtgagagcagagggccagctaagtggtactctcccagagactgtctgactcacgccaccccctccaccttggacacaggacgctgtggtttctgagccaggtacaatgactcctttcggtaagtgcagtggaagctgtacactgcccaggcaaagcgtccgggcagcgtaggcgggcgactcagatcccagccagtggacttagcccctgtttgctcctccgataactggggtgaccttggttaatattcaccagcagcctcccccgttgcccctctggatccactgcttaaatacggacgaggacagggccctgtctcctcagcttcaggcaccaccactgacctgggacagtgaat

SEQ ID NO: 4 - DNA, 392 bp, Homo sapiens
tgctaccagtggaacagccactaaggattctgcagtgagagcagagggccagctaagtggtactctcccagagactgtctgactcacgccaccccctccaccttggacacaggacgctgtggtttctgagccaggtacaatgactcctttcggtaagtgcagtggaagctgtacactgcccaggcaaagcgtccgggcagcgtaggcgggcgactcagatcccagccagtggacttagcccctgtttgctcctccgataactggggtgaccttggttaatattcaccagcagcctcccccgttgcccctctggatccactgcttaaatacggacgaggacagggccctgtctcctcagcttcaggcaccaccactgacctgggacagtgaat

SEQ ID NO: 5 - DNA, 175 bp, Homo sapiens
ttagggctgattgttgagacactggtgaactttgaacctctgtgatttccctgtttgctctgtgcctgatagctttcagtctgctaacaaatctcctttatgcagtttaacctctgtacttccaatggggaggaattggaatcagcctatgggagaagagatagctctaggattc

SEQ ID NO: 6 - protein, 354 aa, Homo sapiens
MLFNLRILLNNAAFRNGHNFMVRNFRCGQPLQNKVQLKGRDLLTLKNFTGEEIKYMLWLSADLKFRIKQKGEYLPLLQGKSLGMIFEKRSTRTRLSTETGFALLGGHPCFLTTQDIHLGVNESLTDTARVLSSMADAVLARVYKQSDLDTLAKEASIPIINGLSDLYHPIQILADYLTLQEHYSSLKGLTLSWIGDGNNILHSIMMSAAKFGMHLQAATPKGYEPDASVTKLAEQYAKENGTKLLLTNDPLEAAHGGNVLITDTWISMGQEEEKKKRLQAFQGYQVTMKTAKVAASDWTFLHCLPRKPEEVDDEVFYSPRSLVFPEAENRKWTIMAVMVSLLTDYSPQLQKPKF

SEQ ID NO: 7 - DNA, 1464 bp, Homo sapiens
aagctgaagggtgatattacctttgctccctcactgcaactgaacacatttcttagtttttaggtggcccccgctggctaacttgctgtggagttttcaagggcatagaatcgtcctttacacaattaaaagaagatgctgtttaatctgaggatcctgttaaacaatgcagcttttagaaatggtcacaacttcatggttcgaaattttcggtgtggacaaccactacaaaataaagtgcagctgaagggccgtgaccttctcactctaaaaaactttaccggagaagaaattaaatatatgctatggctatcagcagatctgaaatttaggataaaacagaaaggagagtatttgcctttattgcaggggaagtccttaggcatgatttttgagaaaagaagtactcgaacaagattgtctacagaaacaggctttgcacttctgggaggacatccttgttttcctaccacacaagatattcatttgggtgtgaatgaaagtctcacggacacggcccgtgtattgtctagcatggcagatgcagtattggctcgagtgtataaacaatcagatttggacacccttgctaaagaagcatccatcccaattatcaatgggctgtcagatttgtaccatcctatccagatcctggctgattacctcacgctccaggaacactatagctctctgaaaggtcttaccctcagctgtttcggggatgggaacaatatcctgcactccatcatgatgagcgcagcgaaattcggaatgcaccttcaggcagctactccaaagggttatgagccggatgctagtgtaaccaagttggcagagcagtatgccaaagagaatggtaccaagctgttgctgacaaatgatccattggaagcagcgcatggaggcaatgtattaattacagacacttggataagcatgggacgagaagaggagaagaaaaagcggctccaagctttccaaggttaccaagttacaatgaagactgctaaagttgctgcctctgactggacatttttacactgcttgcccagaaagccagaagaagtggatgatgaagtcttttattctcctcgatcactagtgttcccagaggcagaaaacagaaagtggacaatcatggctgtcatggtgtccctgctgacagattactcacctcagctccagaagcctaaattttgatgttgtgttacttgtcaagaaagaagcaatgttggtcagtaacagaatgagttggtttatggggaaaagagaagagaatctaaaaaataaaccaatccctaacacgtggtatgggcgaatcgtacgatatgctttgccattgtgaaactttccttaagccttcaatttaagtgctgatgcactgtaatacgtgcttaactttgcttaaactctctaattcccaatttctgagttacatttagatatcatattaactatcatata

SEQ ID NO: 8 - DNA, 1065 bp, Artificial Sequence
  Codon-optimized human OTC coding sequence
atgctgtttaacctgagaatcctgctgaataacgctgcctttaggaacggacataacttcatggtccgcaactttcgctgtggccagcctctccagaacaaagtgcagctgaaggggagggacctgctgaccctgaaaaatttcacaggagaggaaatcaagtacatgctgtggctgtctgccgatctgaagttccggatcaagcagaagggcgaatatctgccactgctccagggcaaaagtctggggatgatcttcgaaaagaggagtactcggaccagactgtcaacagagactggattcgctctgctgggaggacacccatgctttctgaccacacaggacattcatctgggcgtgaacgagtcactgaccgacacagcccgggtgctgagcagcatggccgatgccgtgctggcacgggtctacaaacagagcgacctggataccctggctaaggaagcaagcatccccatcattaatgggctgtccgacctgtatcaccctatccagattctggccgattacctgaccctccaggagcattattctagtctgaaaggcctgacactgagctggattggggacggaaacaatatcctgcactccattatgatgtctgccgctaagtttgggatgcacctccaggcagccacaccaaaaggctacgaacccgatgccagtgtgactaagctggccgaacagtatgctaaagagaacggcactaagctgctgctgaccaatgaccccctggaggctgcacacggaggcaacgtcctgatcactgatacctggatcagcatgggccaggaggaagagaagaagaagcggctccaggccttccagggctaccaggtgacaatgaaaactgccaaggtcgccgcttctgattggacttttctgcattgtctgccccgaaaacctgaagaggtggacgatgaggtcttctattcacctaggagcctggtgtttccagaagccgagaatcgcaagtggacaatcatggccgtgatggtgtccctgctgactgactattccccacagctgcagaagcctaagttttga

SEQ ID NO: 9 - DNA, 261 bp, Bos taurus
tcgctgatcagcctcgactgtgccttctagttgccagccatctgttgtttgcccctcccccgtgccttccttgaccctggaaggtgccactcccactgtcctttcctaataaaatgaggaaattgcatcgcattgtctgagtaggtgtcattctattctggggggtggggtggggcaggacagcaagggggaggattgggaagacaatagcaggcatgctggggatgcggtgggctctatggcttctgaggcggaaagaac

SEQ ID NO: 10 - DNA, 7 bp, Artificial Sequence
  Kozac sequence
cgccacc

SEQ ID NO: 11 - DNA, 87 bp, Artificial sequence
  Simian virus 40
tctaaggtaaatataaaatttttaagtgtataatgtgttaaactactgattctaattgtttctctcttttagattccaacctttgga

SEQ ID NO: 12 - DNA, 550 bp, Homo sapiens
tgagaacttcagggtgagtctatgggacccttgatgttttctttccccttcttttctatggttaagttcatgtcataggaaggggagaagtaacagggtacacatattgaccaaatcagggtaattttgcatttgtaattttaaaaaatgctttcttcttttaatatacttttttgtttatcttatttctaatactttccctaatctctttctttcagggcaataatgatacaatgtatcatgcctctttgcaccattctaaagaataacagtgataatttctgggttaaggcaatagcaatatttctgcatataaatatttctgcatataaattgtaactgatgtaagaggtttcatattgctaatagcagctacaatccagctaccattctgcttttattttatggttgggataaggctggattattctgagtccaagctaggcccttttgctaatcatgttcatacctcttatcttcctcccacagctcctgggcaacgtgctggtctgtgtgctggcccatcactttggcaaagcacgtgagatct

SEQ ID NO: 13 - DNA, 145 bp, adeno-associated virus
ttggccactccctctctgcgcgctcgctcgctcactgaggccgcccgggcaaagcccgggcgtcgggcgacctttggtcgcccggcctcagtgagcgagcgagcgcgcagagagggagtggccaactccatcactaggggttcct

SEQ ID NO: 14 - DNA, 145 bp, adeno-associated virus
aggaacccctagtgatggagttggccactccctctctgcgcgctcgctcgctcactgaggccgggcgaccaaaggtcgcccgacgcccgggctttgcccgggcggcctcagtgagcgagcgagcgcgcagagagggagtggccaa

SEQ ID NO: 15 - DNA, 3872 bp, Artificial sequence
  hOTCenh.hOTCprom.SV40int.hOTCco.BGHpa expression cassette
ttagggctgattgttgagacactggtgaactttgaacctctgtgatttccctgtttgctctgtgcctgatagctttcagtctgctaacaaatctcctttatgcagtttaacctctgtacttccaatggggaggaattggaatcagcctatgggagaagagatagctctaggattcagatctacaagaaagttaaaattgaattagaggaatcatggggtcaacaagagcccctggatgaattctgaggatgaacatcaaagcctgtaaagtaaaacagactccacatgtgacataatcagcagaagctgggtagttgaaatctacccctcaacaagttcattgagatgccctgccttttgagattcagtgaaattgcttttaacttcatcccacttgtgatgcagctccccttttccaatccctctgggagttattggtatcttaacttttttttagttccctctggctttgagctcctgcatctgtagcattaggagggtttgtgagttgctttggcatctcagaaatgctgcctgtactctctagcatggaactgcagacacttcttgatttctccccaagcattaccaatatgagttgtgtgtatggctagcacagttcagtgaagatatggggtcaagctatgggctttatattagcctgtggtttggcctcatctccctcaggctccatgcaaacgttcaatttcactcctgtattatgtggagcgcttttgctctctgaaacctattcaataactggccttgtttgcctcttcaaagatgctttattatgttttttaaattcactctctcccttctcacctctgtacctttgcaagcagttgcttctgcctggaatatcctttccagaatggaagatttggtagaggttgggaaatgtcagtctttcccctcactttatctcacatcattctctgtaagtagaaggaaatggtgacaatatttatttctctactagtattaattatgacatcacaaacatctcggctcctgaggtggccatagttggtctttaaataacactttttggtattccacaaacttctggaaaatatttacttgggtttgctaaagtcatataaattgaccagaagaggcagccctacccctgcccctcctctccttcctcctacccttcctaccttagagggctcccgcttcttcgaagccagacaactttgtctggacctctcctatgggcttgtattatggatatttgtttataaatcataccacctttactgaactgtgaactctgcaaagatgatgtcatcttccctctctgaaacttcagtgcagctcggtatctgatacagaattgactttgaatcacctgatttctaactgaggataaatgaataaatgtgaagttgcagatggccccttagtgatctgaataggctgctaggggaagagcatatggtatccccacttcccacttgtactgactgtcaggtgctgttagaatcaataggcaactatttcttttctttttctttctttctttcttttttttgagacagtgtctctctctgtcacccaggctggagtacagtggtgcaatctgggctcactgcaacctctgtctcccgggttcaagcgactctcatgcctcagcctcccaaatagctgggattacaggtgtgcaccaccacgtctagctaatttttgtatttttagtggagacggggattcaccatgttggccaggctggtctcgaactcctgggctcaagtgatccgcccgcctcagcctcccaaagtgctgggattacaggcgtgagccaccgtgcccggccagcaattatttctttattgaagacttatgtgcaaggcacaaagggagctccaggactgagatatttttactataccttctctatcatcttgcacccccaaaatagcttccagggcacttctttctatttgtttttgtggaaagactggcaattagaggtagaaaagtgaaataaatggaaatagtactactcaggactgtcacatctacatctgtgtttttgcagtgccaatttgcattttctgagtgagttacttctactcaccttcacagcagccggtaccgcagtgccttgcatatattatatcctcaatgagtacttgtcaattgattttgtacatgcgtgtgacagtataaatatattatgaaaaatgaggaggccaggcaataaaagagtcaggatttcttccaaaaaaaatacacagcggtggagcttggcataaagttcaaatgctcctacaccctgccctgcagtatctctaaccaggggactttgataaggaagctgaagggtgatattacctttgctccctcactgcaactgaacacatttcttagtttttaggtggcccccgctggctaacttgctgtggcggccgctctaaggtaaatataaaatttttaagtgtataatgtgttaaactactgattctaattgtttctctcttttagattccaacctttggaactgatctagagaattcgccgccaccatgctgtttaacctgagaatcctgctgaataacgctgcctttaggaacggacataacttcatggtccgcaactttcgctgtggccagcctctccagaacaaagtgcagctgaaggggagggacctgctgaccctgaaaaatttcacaggagaggaaatcaagtacatgctgtggctgtctgccgatctgaagttccggatcaagcagaagggcgaatatctgccactgctccagggcaaaagtctggggatgatcttcgaaaagaggagtactcggaccagactgtcaacagagactggattcgctctgctgggaggacacccatgctttctgaccacacaggacattcatctgggcgtgaacgagtcactgaccgacacagcccgggtgctgagcagcatggccgatgccgtgctggcacgggtctacaaacagagcgacctggataccctggctaaggaagcaagcatccccatcattaatgggctgtccgacctgtatcaccctatccagattctggccgattacctgaccctccaggagcattattctagtctgaaaggcctgacactgagctggattggggacggaaacaatatcctgcactccattatgatgtctgccgctaagtttgggatgcacctccaggcagccacaccaaaaggctacgaacccgatgccagtgtgactaagctggccgaacagtatgctaaagagaacggcactaagctgctgctgaccaatgaccccctggaggctgcacacggaggcaacgtcctgatcactgatacctggatcagcatgggccaggaggaagagaagaagaagcggctccaggccttccagggctaccaggtgacaatgaaaactgccaaggtcgccgcttctgattggacttttctgcattgtctgccccgaaaacctgaagaggtggacgatgaggtcttctattcacctaggagcctggtgtttccagaagccgagaatcgcaagtggacaatcatggccgtgatggtgtccctgctgactgactattccccacagctgcagaagcctaagttttgagatatcgtcgactcgctgatcagcctcgactgtgccttctagttgccagccatctgttgtttgcccctcccccgtgccttccttgaccctggaaggtgccactcccactgtcctttcctaataaaatgaggaaattgcatcgcattgtctgagtaggtgtcattctattctggggggtggggtggggcaggacagcaagggggaggattgggaagacaatagcaggcatgctggggatgcggtgggctctatggcttctgaggcggaaagaac

SEQ ID NO: 16 - DNA, 4250 bp, Artificial sequence
  AAV2-hOTCenh.hOTCprom.SV40int.hOTCco.BGHpa expression cassette
ttggccactccctctctgcgcgctcgctcgctcactgaggccgcccgggcaaagcccgggcgtcgggcgacctttggtcgcccggcctcagtgagcgagcgagcgcgcagagagggagtggccaactccatcactaggggttccttacgtagccatgctctagcgatcgcggtaccttaattaattagggctgattgttgagacactggtgaactttgaacctctgtgatttccctgtttgctctgtgcctgatagctttcagtctgctaacaaatctcctttatgcagtttaacctctgtacttccaatggggaggaattggaatcagcctatgggagaagagatagctctaggattcagatctacaagaaagttaaaattgaattagaggaatcatggggtcaacaagagcccctggatgaattctgaggatgaacatcaaagcctgtaaagtaaaacagactccacatgtgacataatcagcagaagctgggtagttgaaatctacccctcaacaagttcattgagatgccctgccttttgagattcagtgaaattgcttttaacttcatcccacttgtgatgcagctccccttttccaatccctctgggagttattggtatcttaacttttttttagttccctctggctttgagctcctgcatctgtagcattaggagggtttgtgagttgctttggcatctcagaaatgctgcctgtactctctagcatggaactgcagacacttcttgatttctccccaagcattaccaatatgagttgtgtgtatggctagcacagttcagtgaagatatggggtcaagctatgggctttatattagcctgtggtttggcctcatctccctcaggctccatgcaaacgttcaatttcactcctgtattatgtggagcgcttttgctctctgaaacctattcaataactggccttgtttgcctcttcaaagatgctttattatgttttttaaattcactctctcccttctcacctctgtacctttgcaagcagttgcttctgcctggaatatcctttccagaatggaagatttggtagaggttgggaaatgtcagtctttcccctcactttatctcacatcattctctgtaagtagaaggaaatggtgacaatatttatttctctactagtattaattatgacatcacaaacatctcggctcctgaggtggccatagttggtctttaaataacactttttggtattccacaaacttctggaaaatatttacttgggtttgctaaagtcatataaattgaccagaagaggcagccctacccctgcccctcctctccttcctcctacccttcctaccttagagggctcccgcttcttcgaagccagacaactttgtctggacctctcctatgggcttgtattatggatatttgtttataaatcataccacctttactgaactgtgaactctgcaaagatgatgtcatcttccctctctgaaacttcagtgcagctcggtatctgatacagaattgactttgaatcacctgatttctaactgaggataaatgaataaatgtgaagttgcagatggccccttagtgatctgaataggctgctaggggaagagcatatggtatccccacttcccacttgtactgactgtcaggtgctgttagaatcaataggcaactatttcttttctttttctttctttctttcttttttttgagacagtgtctctctctgtcacccaggctggagtacagtggtgcaatctgggctcactgcaacctctgtctcccgggttcaagcgactctcatgcctcagcctcccaaatagctgggattacaggtgtgcaccaccacgtctagctaatttttgtatttttagtggagacggggattcaccatgttggccaggctggtctcgaactcctgggctcaagtgatccgcccgcctcagcctcccaaagtgctgggattacaggcgtgagccaccgtgcccggccagcaattatttctttattgaagacttatgtgcaaggcacaaagggagctccaggactgagatatttttactataccttctctatcatcttgcacccccaaaatagcttccagggcacttctttctatttgtttttgtggaaagactggcaattagaggtagaaaagtgaaataaatggaaatagtactactcaggactgtcacatctacatctgtgtttttgcagtgccaatttgcattttctgagtgagttacttctactcaccttcacagcagccggtaccgcagtgccttgcatatattatatcctcaatgagtacttgtcaattgattttgtacatgcgtgtgacagtataaatatattatgaaaaatgaggaggccaggcaataaaagagtcaggatttcttccaaaaaaaatacacagcggtggagcttggcataaagttcaaatgctcctacaccctgccctgcagtatctctaaccaggggactttgataaggaagctgaagggtgatattacctttgctccctcactgcaactgaacacatttcttagtttttaggtggcccccgctggctaacttgctgtggcggccgctctaaggtaaatataaaatttttaagtgtataatgtgttaaactactgattctaattgtttctctcttttagattccaacctttggaactgatctagagaattcgccgccaccatgctgtttaacctgagaatcctgctgaataacgctgcctttaggaacggacataacttcatggtccgcaactttcgctgtggccagcctctccagaacaaagtgcagctgaaggggagggacctgctgaccctgaaaaatttcacaggagaggaaatcaagtacatgctgtggctgtctgccgatctgaagttccggatcaagcagaagggcgaatatctgccactgctccagggcaaaagtctggggatgatcttcgaaaagaggagtactcggaccagactgtcaacagagactggattcgctctgctgggaggacacccatgctttctgaccacacaggacattcatctgggcgtgaacgagtcactgaccgacacagcccgggtgctgagcagcatggccgatgccgtgctggcacgggtctacaaacagagcgacctggataccctggctaaggaagcaagcatccccatcattaatgggctgtccgacctgtatcaccctatccagattctggccgattacctgaccctccaggagcattattctagtctgaaaggcctgacactgagctggattggggacggaaacaatatcctgcactccattatgatgtctgccgctaagtttgggatgcacctccaggcagccacaccaaaaggctacgaacccgatgccagtgtgactaagctggccgaacagtatgctaaagagaacggcactaagctgctgctgaccaatgaccccctggaggctgcacacggaggcaacgtcctgatcactgatacctggatcagcatgggccaggaggaagagaagaagaagcggctccaggccttccagggctaccaggtgacaatgaaaactgccaaggtcgccgcttctgattggacttttctgcattgtctgccccgaaaacctgaagaggtggacgatgaggtcttctattcacctaggagcctggtgtttccagaagccgagaatcgcaagtggacaatcatggccgtgatggtgtccctgctgactgactattccccacagctgcagaagcctaagttttgagatatcgtcgactcgctgatcagcctcgactgtgccttctagttgccagccatctgttgtttgcccctcccccgtgccttccttgaccctggaaggtgccactcccactgtcctttcctaataaaatgaggaaattgcatcgcattgtctgagtaggtgtcattctattctggggggtggggtggggcaggacagcaagggggaggattgggaagacaatagcaggcatgctggggatgcggtgggctctatggcttctgaggcggaaagaaccagctggggctcgactagactagtcctgcaggtagagcatggctacgtaaggaacccctagtgatggagttggccactccctctctgcgcgctcgctcgctcactgaggccgggcgaccaaaggtcgcccgacgcccgggctttgcccgggcggcctcagtgagcgagcgagcgcgcagagagggagtggccaa

SEQ ID NO: 17 - DNA, 3872 bp, Artificial sequence
  hOTCenh.hAATprom.SV40int.hOTCco.BGHpa expression cassette
ttagggctgattgttgagacactggtgaactttgaacctctgtgatttccctgtttgctctgtgcctgatagctttcagtctgctaacaaatctcctttatgcagtttaacctctgtacttccaatggggaggaattggaatcagcctatgggagaagagatagctctaggattcagatctcccagtcttgtgtctgccgggcaatgagcaaggctccttcctgtccaagctccccgcccctccccagcctactgcctccacccgaagtctacttcctgggtgggcaggaactgggcactgtgcccagggcatgcactgcctccacgcagcaaccctcagagtcctgagctgaaccaagaaggaggagggggtcgggcctccgaggaaggcctagccgctgctgctgccaggaattccaggttggaggggcggcaacctcctgccagccttcaggccactctcctgtgcctgccagaagagacagagcttgaggagagcttgaggagagcaggaaaggtgggacattgctgctgctgctcactcagttccacaggtgggagggacagcagggcttagagtgggggtcattgtgcagatgggaaaacaaaggcccagagaggggaagaaatgcccaggagctaccgagggcaggcgacctcaaccacagcccagtgctggagctgtgagtggatgtagagcagcggaatatccattcagccagctcaggggaaggacaggggccctgaagccaggggatggagctgcagggaagggagctcagagagaaggggaggggagtctgagctcagtttcccgctgcctgaaaggagggtggtacctactcccttcacagggtaactgaatgagagactgcctggaggaaagctcttcaagtgtggcccaccccaccccagtgacaccagcccctgacacgggggagggagggcagcatcaggaggggctttctgggcacacccagtacccgtctctgagctttccttgaactgttgcattttaatcctcacagcagctcaacaaggtacataccgtcaccatccccattttacagatagggaaattgaggctcggagcggttaaacaactcacctgaggcctcacagccagtaagtgggttccctggtctgaatgtgtgtgctggaggatcctgtgggtcactcgcctggtagagccccaaggtggaggcataaatgggactggtgaatgacagaaggggcaaaaatgcactcatccattcactctgcaagtatctacggcacgtacgccagctcccaagcaggtttgcgggttgcacagcgggcgatgcaatctgatttaggcttttaaagggattgcaatcaagtggggccccactagcctcaaccctgtacctcccctcccctccacccccagcagtctccaaaggcctccaacaaccccagagtgggggccatgtatccaaagaaactccaagctgtatacggatcacactggttttccaggagcaaaaacagaaacaggcctgaggctggtcaaaattgaacctcctcctgctctgagcagcctggggggcagactaagcagagggctgtgcagacccacataaagagcctactgtgtgccaggcacttcacccgaggcacttcacaagcatgcttgggaatgaaacttccaactctttgggatgcaggtgaaacagttcctggttcagagaggtgaagcggcctgcctgaggcagcacagctcttctttacagatgtgcttccccacctctaccctgtctcacggccccccatgccagcctgacggttgtgtctgcctcagtcatgctccatttttccatcgggaccatcaagagggtgtttgtgtctaaggctgactgggtaactttggatgagcggtctctccgctctgagcctgtttcctcatctgtcaaatgggctctaacccactctgatctcccagggcggcagtaagtcttcagcatcaggcattttggggtgactcagtaaatggtagatcttgctaccagtggaacagccactaaggattctgcagtgagagcagagggccagctaagtggtactctcccagagactgtctgactcacgccaccccctccaccttggacacaggacgctgtggtttctgagccaggtacaatgactcctttcggtaagtgcagtggaagctgtacactgcccaggcaaagcgtccgggcagcgtaggcgggcgactcagatcccagccagtggacttagcccctgtttgctcctccgataactggggtgaccttggttaatattcaccagcagcctcccccgttgcccctctggatccactgcttaaatacggacgaggacagggccctgtctcctcagcttcaggcaccaccactgacctgggacagtgaatgcggccgctctaaggtaaatataaaatttttaagtgtataatgtgttaaactactgattctaattgtttctctcttttagattccaacctttggaactgatctagagaattcgccgccaccatgctgtttaacctgagaatcctgctgaataacgctgcctttaggaacggacataacttcatggtccgcaactttcgctgtggccagcctctccagaacaaagtgcagctgaaggggagggacctgctgaccctgaaaaatttcacaggagaggaaatcaagtacatgctgtggctgtctgccgatctgaagttccggatcaagcagaagggcgaatatctgccactgctccagggcaaaagtctggggatgatcttcgaaaagaggagtactcggaccagactgtcaacagagactggattcgctctgctgggaggacacccatgctttctgaccacacaggacattcatctgggcgtgaacgagtcactgaccgacacagcccgggtgctgagcagcatggccgatgccgtgctggcacgggtctacaaacagagcgacctggataccctggctaaggaagcaagcatccccatcattaatgggctgtccgacctgtatcaccctatccagattctggccgattacctgaccctccaggagcattattctagtctgaaaggcctgacactgagctggattggggacggaaacaatatcctgcactccattatgatgtctgccgctaagtttgggatgcacctccaggcagccacaccaaaaggctacgaacccgatgccagtgtgactaagctggccgaacagtatgctaaagagaacggcactaagctgctgctgaccaatgaccccctggaggctgcacacggaggcaacgtcctgatcactgatacctggatcagcatgggccaggaggaagagaagaagaagcggctccaggccttccagggctaccaggtgacaatgaaaactgccaaggtcgccgcttctgattggacttttctgcattgtctgccccgaaaacctgaagaggtggacgatgaggtcttctattcacctaggagcctggtgtttccagaagccgagaatcgcaagtggacaatcatggccgtgatggtgtccctgctgactgactattccccacagctgcagaagcctaagttttgagatatcgtcgactcgctgatcagcctcgactgtgccttctagttgccagccatctgttgtttgcccctcccccgtgccttccttgaccctggaaggtgccactcccactgtcctttcctaataaaatgaggaaattgcatcgcattgtctgagtaggtgtcattctattctggggggtggggtggggcaggacagcaagggggaggattgggaagacaatagcaggcatgctggggatgcggtgggctctatggcttctgaggcggaaagaac

SEQ ID NO: 18 - DNA, 4250 bp, Artificial sequence
  AAV2-hOTCenh.hAATprom.SV40int.hOTCco.BGHpa expression cassette
ttggccactccctctctgcgcgctcgctcgctcactgaggccgcccgggcaaagcccgggcgtcgggcgacctttggtcgcccggcctcagtgagcgagcgagcgcgcagagagggagtggccaactccatcactaggggttccttacgtagccatgctctagcgatcgcggtaccttaattaattagggctgattgttgagacactggtgaactttgaacctctgtgatttccctgtttgctctgtgcctgatagctttcagtctgctaacaaatctcctttatgcagtttaacctctgtacttccaatggggaggaattggaatcagcctatgggagaagagatagctctaggattcagatctcccagtcttgtgtctgccgggcaatgagcaaggctccttcctgtccaagctccccgcccctccccagcctactgcctccacccgaagtctacttcctgggtgggcaggaactgggcactgtgcccagggcatgcactgcctccacgcagcaaccctcagagtcctgagctgaaccaagaaggaggagggggtcgggcctccgaggaaggcctagccgctgctgctgccaggaattccaggttggaggggcggcaacctcctgccagccttcaggccactctcctgtgcctgccagaagagacagagcttgaggagagcttgaggagagcaggaaaggtgggacattgctgctgctgctcactcagttccacaggtgggagggacagcagggcttagagtgggggtcattgtgcagatgggaaaacaaaggcccagagaggggaagaaatgcccaggagctaccgagggcaggcgacctcaaccacagcccagtgctggagctgtgagtggatgtagagcagcggaatatccattcagccagctcaggggaaggacaggggccctgaagccaggggatggagctgcagggaagggagctcagagagaaggggaggggagtctgagctcagtttcccgctgcctgaaaggagggtggtacctactcccttcacagggtaactgaatgagagactgcctggaggaaagctcttcaagtgtggcccaccccaccccagtgacaccagcccctgacacgggggagggagggcagcatcaggaggggctttctgggcacacccagtacccgtctctgagctttccttgaactgttgcattttaatcctcacagcagctcaacaaggtacataccgtcaccatccccattttacagatagggaaattgaggctcggagcggttaaacaactcacctgaggcctcacagccagtaagtgggttccctggtctgaatgtgtgtgctggaggatcctgtgggtcactcgcctggtagagccccaaggtggaggcataaatgggactggtgaatgacagaaggggcaaaaatgcactcatccattcactctgcaagtatctacggcacgtacgccagctcccaagcaggtttgcgggttgcacagcgggcgatgcaatctgatttaggcttttaaagggattgcaatcaagtggggccccactagcctcaaccctgtacctcccctcccctccacccccagcagtctccaaaggcctccaacaaccccagagtgggggccatgtatccaaagaaactccaagctgtatacggatcacactggttttccaggagcaaaaacagaaacaggcctgaggctggtcaaaattgaacctcctcctgctctgagcagcctggggggcagactaagcagagggctgtgcagacccacataaagagcctactgtgtgccaggcacttcacccgaggcacttcacaagcatgcttgggaatgaaacttccaactctttgggatgcaggtgaaacagttcctggttcagagaggtgaagcggcctgcctgaggcagcacagctcttctttacagatgtgcttccccacctctaccctgtctcacggccccccatgccagcctgacggttgtgtctgcctcagtcatgctccatttttccatcgggaccatcaagagggtgtttgtgtctaaggctgactgggtaactttggatgagcggtctctccgctctgagcctgtttcctcatctgtcaaatgggctctaacccactctgatctcccagggcggcagtaagtcttcagcatcaggcattttggggtgactcagtaaatggtagatcttgctaccagtggaacagccactaaggattctgcagtgagagcagagggccagctaagtggtactctcccagagactgtctgactcacgccaccccctccaccttggacacaggacgctgtggtttctgagccaggtacaatgactcctttcggtaagtgcagtggaagctgtacactgcccaggcaaagcgtccgggcagcgtaggcgggcgactcagatcccagccagtggacttagcccctgtttgctcctccgataactggggtgaccttggttaatattcaccagcagcctcccccgttgcccctctggatccactgcttaaatacggacgaggacagggccctgtctcctcagcttcaggcaccaccactgacctgggacagtgaatgcggccgctctaaggtaaatataaaatttttaagtgtataatgtgttaaactactgattctaattgtttctctcttttagattccaacctttggaactgatctagagaattcgccgccaccatgctgtttaacctgagaatcctgctgaataacgctgcctttaggaacggacataacttcatggtccgcaactttcgctgtggccagcctctccagaacaaagtgcagctgaaggggagggacctgctgaccctgaaaaatttcacaggagaggaaatcaagtacatgctgtggctgtctgccgatctgaagttccggatcaagcagaagggcgaatatctgccactgctccagggcaaaagtctggggatgatcttcgaaaagaggagtactcggaccagactgtcaacagagactggattcgctctgctgggaggacacccatgctttctgaccacacaggacattcatctgggcgtgaacgagtcactgaccgacacagcccgggtgctgagcagcatggccgatgccgtgctggcacgggtctacaaacagagcgacctggataccctggctaaggaagcaagcatccccatcattaatgggctgtccgacctgtatcaccctatccagattctggccgattacctgaccctccaggagcattattctagtctgaaaggcctgacactgagctggattggggacggaaacaatatcctgcactccattatgatgtctgccgctaagtttgggatgcacctccaggcagccacaccaaaaggctacgaacccgatgccagtgtgactaagctggccgaacagtatgctaaagagaacggcactaagctgctgctgaccaatgaccccctggaggctgcacacggaggcaacgtcctgatcactgatacctggatcagcatgggccaggaggaagagaagaagaagcggctccaggccttccagggctaccaggtgacaatgaaaactgccaaggtcgccgcttctgattggacttttctgcattgtctgccccgaaaacctgaagaggtggacgatgaggtcttctattcacctaggagcctggtgtttccagaagccgagaatcgcaagtggacaatcatggccgtgatggtgtccctgctgactgactattccccacagctgcagaagcctaagttttgagatatcgtcgactcgctgatcagcctcgactgtgccttctagttgccagccatctgttgtttgcccctcccccgtgccttccttgaccctggaaggtgccactcccactgtcctttcctaataaaatgaggaaattgcatcgcattgtctgagtaggtgtcattctattctggggggtggggtggggcaggacagcaagggggaggattgggaagacaatagcaggcatgctggggatgcggtgggctctatggcttctgaggcggaaagaaccagctggggctcgactagactagtcctgcaggtagagcatggctacgtaaggaacccctagtgatggagttggccactccctctctgcgcgctcgctcgctcactgaggccgggcgaccaaaggtcgcccgacgcccgggctttgcccgggcggcctcagtgagcgagcgagcgcgcagagagggagtggccaa

SEQ ID NO: 19 - DNA, 2604 bp, Artificial sequence
  2hOTCenh.hOTCprom.SV40int.hOTCco.BGHpa expression cassette
ttagggctgattgttgagacactggtgaactttgaacctctgtgatttccctgtttgctctgtgcctgatagctttcagtctgctaacaaatctcctttatgcagtttaacctctgtacttccaatggggaggaattggaatcagcctatgggagaagagatagctctaggattcttagggctgattgttgagacactggtgaactttgaacctctgtgatttccctgtttgctctgtgcctgatagctttcagtctgctaacaaatctcctttatgcagtttaacctctgtacttccaatggggaggaattggaatcagcctatgggagaagagatagctctaggattcagatctcaagcgactctcatgcctcagcctcccaaatagctgggattacaggtgtgcaccaccacgtctagctaatttttgtatttttagtggagacggggattcatcatgttggccaggctggtctcgaactcctgggctcaagtgatccgcccgcctcagcctcccaaagtgctgggattataggcgtgagccaccatgcccggccagcaattatttctttattgaagacttatgtgcaaggcacaaagggagctccaggactgagatatttttactataccttctctatcatcttgcacccccaaaatagcttccagggcacttctatttgtttttgtggaaagactggcaattagaggtagaaaagtgaaataaatggaaatagtactactcagggctgtcacatctacatctgtgtttttgcagtgccaatttgcattttctgagtgagttacttctactcaccttcacagcagccagtaccgcagtgccttgcatatattatatcctcaatgagtacttgtcaattgattttgtacatgcgtgtgacagtataaatatattatgaaaaatgaggaggccaggcaataaaagagtcaggatttcttccaaaaaaaatacacagcggtggagcttggcataaagttcaaatgctcctacaccctgccctgcagtatctctaaccaggggactttgataaggaagctgaagggtgatattacctttgctccctcactgcaactgaacacatttcttagtttttaggtggcccccgctggctaacttgctgtggcggccgctctaaggtaaatataaaatttttaagtgtataatgtgttaaactactgattctaattgtttctctcttttagattccaacctttggaactgatctagagaattcgccgccaccatgctgtttaacctgagaatcctgctgaataacgctgcctttaggaacggacataacttcatggtccgcaactttcgctgtggccagcctctccagaacaaagtgcagctgaaggggagggacctgctgaccctgaaaaatttcacaggagaggaaatcaagtacatgctgtggctgtctgccgatctgaagttccggatcaagcagaagggcgaatatctgccactgctccagggcaaaagtctggggatgatcttcgaaaagaggagtactcggaccagactgtcaacagagactggattcgctctgctgggaggacacccatgctttctgaccacacaggacattcatctgggcgtgaacgagtcactgaccgacacagcccgggtgctgagcagcatggccgatgccgtgctggcacgggtctacaaacagagcgacctggataccctggctaaggaagcaagcatccccatcattaatgggctgtccgacctgtatcaccctatccagattctggccgattacctgaccctccaggagcattattctagtctgaaaggcctgacactgagctggattggggacggaaacaatatcctgcactccattatgatgtctgccgctaagtttgggatgcacctccaggcagccacaccaaaaggctacgaacccgatgccagtgtgactaagctggccgaacagtatgctaaagagaacggcactaagctgctgctgaccaatgaccccctggaggctgcacacggaggcaacgtcctgatcactgatacctggatcagcatgggccaggaggaagagaagaagaagcggctccaggccttccagggctaccaggtgacaatgaaaactgccaaggtcgccgcttctgattggacttttctgcattgtctgccccgaaaacctgaagaggtggacgatgaggtcttctattcacctaggagcctggtgtttccagaagccgagaatcgcaagtggacaatcatggccgtgatggtgtccctgctgactgactattccccacagctgcagaagcctaagttttgagatatcgtcgactcgctgatcagcctcgactgtgccttctagttgccagccatctgttgtttgcccctcccccgtgccttccttgaccctggaaggtgccactcccactgtcctttcctaataaaatgaggaaattgcatcgcattgtctgagtaggtgtcattctattctggggggtggggtggggcaggacagcaagggggaggattgggaagacaatagcaggcatgctggggatgcggtgggctctatggcttctgaggcggaaagaac

SEQ ID NO: 20 - DNA, 2982 bp, Artificial sequence
  AAV2-2hOTCenh.hOTCprom.SV40int.hOTCco.BGHpa expression cassette
ttggccactccctctctgcgcgctcgctcgctcactgaggccgcccgggcaaagcccgggcgtcgggcgacctttggtcgcccggcctcagtgagcgagcgagcgcgcagagagggagtggccaactccatcactaggggttccttacgtagccatgctctagcgatcgcggtaccttaattaattagggctgattgttgagacactggtgaactttgaacctctgtgatttccctgtttgctctgtgcctgatagctttcagtctgctaacaaatctcctttatgcagtttaacctctgtacttccaatggggaggaattggaatcagcctatgggagaagagatagctctaggattcttagggctgattgttgagacactggtgaactttgaacctctgtgatttccctgtttgctctgtgcctgatagctttcagtctgctaacaaatctcctttatgcagtttaacctctgtacttccaatggggaggaattggaatcagcctatgggagaagagatagctctaggattcagatctcaagcgactctcatgcctcagcctcccaaatagctgggattacaggtgtgcaccaccacgtctagctaatttttgtatttttagtggagacggggattcatcatgttggccaggctggtctcgaactcctgggctcaagtgatccgcccgcctcagcctcccaaagtgctgggattataggcgtgagccaccatgcccggccagcaattatttctttattgaagacttatgtgcaaggcacaaagggagctccaggactgagatatttttactataccttctctatcatcttgcacccccaaaatagcttccagggcacttctatttgtttttgtggaaagactggcaattagaggtagaaaagtgaaataaatggaaatagtactactcagggctgtcacatctacatctgtgtttttgcagtgccaatttgcattttctgagtgagttacttctactcaccttcacagcagccagtaccgcagtgccttgcatatattatatcctcaatgagtacttgtcaattgattttgtacatgcgtgtgacagtataaatatattatgaaaaatgaggaggccaggcaataaaagagtcaggatttcttccaaaaaaaatacacagcggtggagcttggcataaagttcaaatgctcctacaccctgccctgcagtatctctaaccaggggactttgataaggaagctgaagggtgatattacctttgctccctcactgcaactgaacacatttcttagtttttaggtggcccccgctggctaacttgctgtggcggccgctctaaggtaaatataaaatttttaagtgtataatgtgttaaactactgattctaattgtttctctcttttagattccaacctttggaactgatctagagaattcgccgccaccatgctgtttaacctgagaatcctgctgaataacgctgcctttaggaacggacataacttcatggtccgcaactttcgctgtggccagcctctccagaacaaagtgcagctgaaggggagggacctgctgaccctgaaaaatttcacaggagaggaaatcaagtacatgctgtggctgtctgccgatctgaagttccggatcaagcagaagggcgaatatctgccactgctccagggcaaaagtctggggatgatcttcgaaaagaggagtactcggaccagactgtcaacagagactggattcgctctgctgggaggacacccatgctttctgaccacacaggacattcatctgggcgtgaacgagtcactgaccgacacagcccgggtgctgagcagcatggccgatgccgtgctggcacgggtctacaaacagagcgacctggataccctggctaaggaagcaagcatccccatcattaatgggctgtccgacctgtatcaccctatccagattctggccgattacctgaccctccaggagcattattctagtctgaaaggcctgacactgagctggattggggacggaaacaatatcctgcactccattatgatgtctgccgctaagtttgggatgcacctccaggcagccacaccaaaaggctacgaacccgatgccagtgtgactaagctggccgaacagtatgctaaagagaacggcactaagctgctgctgaccaatgaccccctggaggctgcacacggaggcaacgtcctgatcactgatacctggatcagcatgggccaggaggaagagaagaagaagcggctccaggccttccagggctaccaggtgacaatgaaaactgccaaggtcgccgcttctgattggacttttctgcattgtctgccccgaaaacctgaagaggtggacgatgaggtcttctattcacctaggagcctggtgtttccagaagccgagaatcgcaagtggacaatcatggccgtgatggtgtccctgctgactgactattccccacagctgcagaagcctaagttttgagatatcgtcgactcgctgatcagcctcgactgtgccttctagttgccagccatctgttgtttgcccctcccccgtgccttccttgaccctggaaggtgccactcccactgtcctttcctaataaaatgaggaaattgcatcgcattgtctgagtaggtgtcattctattctggggggtggggtggggcaggacagcaagggggaggattgggaagacaatagcaggcatgctggggatgcggtgggctctatggcttctgaggcggaaagaaccagctggggctcgactagactagtcctgcaggtagagcatggctacgtaaggaacccctagtgatggagttggccactccctctctgcgcgctcgctcgctcactgaggccgggcgaccaaaggtcgcccgacgcccgggctttgcccgggcggcctcagtgagcgagcgagcgcgcagagagggagtggccaa

SEQ ID NO: 21 - DNA, 3050 bp, Artificial sequence
  2hOTCenh.hOTCprom.betagint.hOTCco.BGHpa expression cassette
ttagggctgattgttgagacactggtgaactttgaacctctgtgatttccctgtttgctctgtgcctgatagctttcagtctgctaacaaatctcctttatgcagtttaacctctgtacttccaatggggaggaattggaatcagcctatgggagaagagatagctctaggattcttagggctgattgttgagacactggtgaactttgaacctctgtgatttccctgtttgctctgtgcctgatagctttcagtctgctaacaaatctcctttatgcagtttaacctctgtacttccaatggggaggaattggaatcagcctatgggagaagagatagctctaggattcagatctcaagcgactctcatgcctcagcctcccaaatagctgggattacaggtgtgcaccaccacgtctagctaatttttgtatttttagtggagacggggattcatcatgttggccaggctggtctcgaactcctgggctcaagtgatccgcccgcctcagcctcccaaagtgctgggattataggcgtgagccaccatgcccggccagcaattatttctttattgaagacttatgtgcaaggcacaaagggagctccaggactgagatatttttactataccttctctatcatcttgcacccccaaaatagcttccagggcacttctatttgtttttgtggaaagactggcaattagaggtagaaaagtgaaataaatggaaatagtactactcagggctgtcacatctacatctgtgtttttgcagtgccaatttgcattttctgagtgagttacttctactcaccttcacagcagccagtaccgcagtgccttgcatatattatatcctcaatgagtacttgtcaattgattttgtacatgcgtgtgacagtataaatatattatgaaaaatgaggaggccaggcaataaaagagtcaggatttcttccaaaaaaaatacacagcggtggagcttggcataaagttcaaatgctcctacaccctgccctgcagtatctctaaccaggggactttgataaggaagctgaagggtgatattacctttgctccctcactgcaactgaacacatttcttagtttttaggtggcccccgctggctaacttgctgtggcggccgctgagaacttcagggtgagtctatgggacccttgatgttttctttccccttcttttctatggttaagttcatgtcataggaaggggagaagtaacagggtacacatattgaccaaatcagggtaattttgcatttgtaattttaaaaaatgctttcttcttttaatatacttttttgtttatcttatttctaatactttccctaatctctttctttcagggcaataatgatacaatgtatcatgcctctttgcaccattctaaagaataacagtgataatttctgggttaaggcaatagcaatatttctgcatataaatatttctgcatataaattgtaactgatgtaagaggtttcatattgctaatagcagctacaatccagctaccattctgcttttattttatggttgggataaggctggattattctgagtccaagctaggcccttttgctaatcatgttcatacctcttatcttcctcccacagctcctgggcaacgtgctggtctgtgtgctggcccatcactttggcaaagcacgtggaattcgccgccaccatgctgtttaacctgagaatcctgctgaataacgctgcctttaggaacggacataacttcatggtccgcaactttcgctgtggccagcctctccagaacaaagtgcagctgaaggggagggacctgctgaccctgaaaaatttcacaggagaggaaatcaagtacatgctgtggctgtctgccgatctgaagttccggatcaagcagaagggcgaatatctgccactgctccagggcaaaagtctggggatgatcttcgaaaagaggagtactcggaccagactgtcaacagagactggattcgctctgctgggaggacacccatgctttctgaccacacaggacattcatctgggcgtgaacgagtcactgaccgacacagcccgggtgctgagcagcatggccgatgccgtgctggcacgggtctacaaacagagcgacctggataccctggctaaggaagcaagcatccccatcattaatgggctgtccgacctgtatcaccctatccagattctggccgattacctgaccctccaggagcattattctagtctgaaaggcctgacactgagctggattggggacggaaacaatatcctgcactccattatgatgtctgccgctaagtttgggatgcacctccaggcagccacaccaaaaggctacgaacccgatgccagtgtgactaagctggccgaacagtatgctaaagagaacggcactaagctgctgctgaccaatgaccccctggaggctgcacacggaggcaacgtcctgatcactgatacctggatcagcatgggccaggaggaagagaagaagaagcggctccaggccttccagggctaccaggtgacaatgaaaactgccaaggtcgccgcttctgattggacttttctgcattgtctgccccgaaaacctgaagaggtggacgatgaggtcttctattcacctaggagcctggtgtttccagaagccgagaatcgcaagtggacaatcatggccgtgatggtgtccctgctgactgactattccccacagctgcagaagcctaagttttgagatatcgtcgactcgctgatcagcctcgactgtgccttctagttgccagccatctgttgtttgcccctcccccgtgccttccttgaccctggaaggtgccactcccactgtcctttcctaataaaatgaggaaattgcatcgcattgtctgagtaggtgtcattctattctggggggtggggtggggcaggacagcaagggggaggattgggaagacaatagcaggcatgctggggatgcggtgggctctatggcttctgaggcggaaagaac

SEQ ID NO: 22 - DNA, 3428 bp, Artificial sequence
  AAV2-2hOTCenh.hOTCprom.beta gint.hOTCco.BGHpa expression cassette
ttggccactccctctctgcgcgctcgctcgctcactgaggccgcccgggcaaagcccgggcgtcgggcgacctttggtcgcccggcctcagtgagcgagcgagcgcgcagagagggagtggccaactccatcactaggggttccttacgtagccatgctctagcgatcgcggtaccttaattaattagggctgattgttgagacactggtgaactttgaacctctgtgatttccctgtttgctctgtgcctgatagctttcagtctgctaacaaatctcctttatgcagtttaacctctgtacttccaatggggaggaattggaatcagcctatgggagaagagatagctctaggattcttagggctgattgttgagacactggtgaactttgaacctctgtgatttccctgtttgctctgtgcctgatagctttcagtctgctaacaaatctcctttatgcagtttaacctctgtacttccaatggggaggaattggaatcagcctatgggagaagagatagctctaggattcagatctcaagcgactctcatgcctcagcctcccaaatagctgggattacaggtgtgcaccaccacgtctagctaatttttgtatttttagtggagacggggattcatcatgttggccaggctggtctcgaactcctgggctcaagtgatccgcccgcctcagcctcccaaagtgctgggattataggcgtgagccaccatgcccggccagcaattatttctttattgaagacttatgtgcaaggcacaaagggagctccaggactgagatatttttactataccttctctatcatcttgcacccccaaaatagcttccagggcacttctatttgtttttgtggaaagactggcaattagaggtagaaaagtgaaataaatggaaatagtactactcagggctgtcacatctacatctgtgtttttgcagtgccaatttgcattttctgagtgagttacttctactcaccttcacagcagccagtaccgcagtgccttgcatatattatatcctcaatgagtacttgtcaattgattttgtacatgcgtgtgacagtataaatatattatgaaaaatgaggaggccaggcaataaaagagtcaggatttcttccaaaaaaaatacacagcggtggagcttggcataaagttcaaatgctcctacaccctgccctgcagtatctctaaccaggggactttgataaggaagctgaagggtgatattacctttgctccctcactgcaactgaacacatttcttagtttttaggtggcccccgctggctaacttgctgtggcggccgctgagaacttcagggtgagtctatgggacccttgatgttttctttccccttcttttctatggttaagttcatgtcataggaaggggagaagtaacagggtacacatattgaccaaatcagggtaattttgcatttgtaattttaaaaaatgctttcttcttttaatatacttttttgtttatcttatttctaatactttccctaatctctttctttcagggcaataatgatacaatgtatcatgcctctttgcaccattctaaagaataacagtgataatttctgggttaaggcaatagcaatatttctgcatataaatatttctgcatataaattgtaactgatgtaagaggtttcatattgctaatagcagctacaatccagctaccattctgcttttattttatggttgggataaggctggattattctgagtccaagctaggcccttttgctaatcatgttcatacctcttatcttcctcccacagctcctgggcaacgtgctggtctgtgtgctggcccatcactttggcaaagcacgtggaattcgccgccaccatgctgtttaacctgagaatcctgctgaataacgctgcctttaggaacggacataacttcatggtccgcaactttcgctgtggccagcctctccagaacaaagtgcagctgaaggggagggacctgctgaccctgaaaaatttcacaggagaggaaatcaagtacatgctgtggctgtctgccgatctgaagttccggatcaagcagaagggcgaatatctgccactgctccagggcaaaagtctggggatgatcttcgaaaagaggagtactcggaccagactgtcaacagagactggattcgctctgctgggaggacacccatgctttctgaccacacaggacattcatctgggcgtgaacgagtcactgaccgacacagcccgggtgctgagcagcatggccgatgccgtgctggcacgggtctacaaacagagcgacctggataccctggctaaggaagcaagcatccccatcattaatgggctgtccgacctgtatcaccctatccagattctggccgattacctgaccctccaggagcattattctagtctgaaaggcctgacactgagctggattggggacggaaacaatatcctgcactccattatgatgtctgccgctaagtttgggatgcacctccaggcagccacaccaaaaggctacgaacccgatgccagtgtgactaagctggccgaacagtatgctaaagagaacggcactaagctgctgctgaccaatgaccccctggaggctgcacacggaggcaacgtcctgatcactgatacctggatcagcatgggccaggaggaagagaagaagaagcggctccaggccttccagggctaccaggtgacaatgaaaactgccaaggtcgccgcttctgattggacttttctgcattgtctgccccgaaaacctgaagaggtggacgatgaggtcttctattcacctaggagcctggtgtttccagaagccgagaatcgcaagtggacaatcatggccgtgatggtgtccctgctgactgactattccccacagctgcagaagcctaagttttgagatatcgtcgactcgctgatcagcctcgactgtgccttctagttgccagccatctgttgtttgcccctcccccgtgccttccttgaccctggaaggtgccactcccactgtcctttcctaataaaatgaggaaattgcatcgcattgtctgagtaggtgtcattctattctggggggtggggtggggcaggacagcaagggggaggattgggaagacaatagcaggcatgctggggatgcggtgggctctatggcttctgaggcggaaagaaccagctggggctcgactagactagtcctgcaggtagagcatggctacgtaaggaacccctagtgatggagttggccactccctctctgcgcgctcgctcgctcactgaggccgggcgaccaaaggtcgcccgacgcccgggctttgcccgggcggcctcagtgagcgagcgagcgcgcagagagggagtggccaa

SEQ ID NO: 23 - DNA, 2207 bp, Artificial sequence
  2hOTCenh.hAATprom.SV40int.hOTCco.BGHpa expression cassette
ttagggctgattgttgagacactggtgaactttgaacctctgtgatttccctgtttgctctgtgcctgatagctttcagtctgctaacaaatctcctttatgcagtttaacctctgtacttccaatggggaggaattggaatcagcctatgggagaagagatagctctaggattcttagggctgattgttgagacactggtgaactttgaacctctgtgatttccctgtttgctctgtgcctgatagctttcagtctgctaacaaatctcctttatgcagtttaacctctgtacttccaatggggaggaattggaatcagcctatgggagaagagatagctctaggattcagatcttgctaccagtggaacagccactaaggattctgcagtgagagcagagggccagctaagtggtactctcccagagactgtctgactcacgccaccccctccaccttggacacaggacgctgtggtttctgagccaggtacaatgactcctttcggtaagtgcagtggaagctgtacactgcccaggcaaagcgtccgggcagcgtaggcgggcgactcagatcccagccagtggacttagcccctgtttgctcctccgataactggggtgaccttggttaatattcaccagcagcctcccccgttgcccctctggatccactgcttaaatacggacgaggacagggccctgtctcctcagcttcaggcaccaccactgacctgggacagtgaatgcggccgctctaaggtaaatataaaatttttaagtgtataatgtgttaaactactgattctaattgtttctctcttttagattccaacctttggaactgatctagagaattcgccgccaccatgctgtttaacctgagaatcctgctgaataacgctgcctttaggaacggacataacttcatggtccgcaactttcgctgtggccagcctctccagaacaaagtgcagctgaaggggagggacctgctgaccctgaaaaatttcacaggagaggaaatcaagtacatgctgtggctgtctgccgatctgaagttccggatcaagcagaagggcgaatatctgccactgctccagggcaaaagtctggggatgatcttcgaaaagaggagtactcggaccagactgtcaacagagactggattcgctctgctgggaggacacccatgctttctgaccacacaggacattcatctgggcgtgaacgagtcactgaccgacacagcccgggtgctgagcagcatggccgatgccgtgctggcacgggtctacaaacagagcgacctggataccctggctaaggaagcaagcatccccatcattaatgggctgtccgacctgtatcaccctatccagattctggccgattacctgaccctccaggagcattattctagtctgaaaggcctgacactgagctggattggggacggaaacaatatcctgcactccattatgatgtctgccgctaagtttgggatgcacctccaggcagccacaccaaaaggctacgaacccgatgccagtgtgactaagctggccgaacagtatgctaaagagaacggcactaagctgctgctgaccaatgaccccctggaggctgcacacggaggcaacgtcctgatcactgatacctggatcagcatgggccaggaggaagagaagaagaagcggctccaggccttccagggctaccaggtgacaatgaaaactgccaaggtcgccgcttctgattggacttttctgcattgtctgccccgaaaacctgaagaggtggacgatgaggtcttctattcacctaggagcctggtgtttccagaagccgagaatcgcaagtggacaatcatggccgtgatggtgtccctgctgactgactattccccacagctgcagaagcctaagttttgagatatcgtcgactcgctgatcagcctcgactgtgccttctagttgccagccatctgttgtttgcccctcccccgtgccttccttgaccctggaaggtgccactcccactgtcctttcctaataaaatgaggaaattgcatcgcattgtctgagtaggtgtcattctattctggggggtggggtggggcaggacagcaagggggaggattgggaagacaatagcaggcatgctggggatgcggtgggctctatggcttctgaggcggaaagaac

SEQ ID NO: 24 - DNA, 2585 bp, Artificial sequence
  AAV2-2hOTCenh.hAATprom.SV40int.hOTCco.BGHpa expression cassette
ttggccactccctctctgcgcgctcgctcgctcactgaggccgcccgggcaaagcccgggcgtcgggcgacctttggtcgcccggcctcagtgagcgagcgagcgcgcagagagggagtggccaactccatcactaggggttccttacgtagccatgctctagcgatcgcggtaccttaattaattagggctgattgttgagacactggtgaactttgaacctctgtgatttccctgtttgctctgtgcctgatagctttcagtctgctaacaaatctcctttatgcagtttaacctctgtacttccaatggggaggaattggaatcagcctatgggagaagagatagctctaggattcttagggctgattgttgagacactggtgaactttgaacctctgtgatttccctgtttgctctgtgcctgatagctttcagtctgctaacaaatctcctttatgcagtttaacctctgtacttccaatggggaggaattggaatcagcctatgggagaagagatagctctaggattcagatcttgctaccagtggaacagccactaaggattctgcagtgagagcagagggccagctaagtggtactctcccagagactgtctgactcacgccaccccctccaccttggacacaggacgctgtggtttctgagccaggtacaatgactcctttcggtaagtgcagtggaagctgtacactgcccaggcaaagcgtccgggcagcgtaggcgggcgactcagatcccagccagtggacttagcccctgtttgctcctccgataactggggtgaccttggttaatattcaccagcagcctcccccgttgcccctctggatccactgcttaaatacggacgaggacagggccctgtctcctcagcttcaggcaccaccactgacctgggacagtgaatgcggccgctctaaggtaaatataaaatttttaagtgtataatgtgttaaactactgattctaattgtttctctcttttagattccaacctttggaactgatctagagaattcgccgccaccatgctgtttaacctgagaatcctgctgaataacgctgcctttaggaacggacataacttcatggtccgcaactttcgctgtggccagcctctccagaacaaagtgcagctgaaggggagggacctgctgaccctgaaaaatttcacaggagaggaaatcaagtacatgctgtggctgtctgccgatctgaagttccggatcaagcagaagggcgaatatctgccactgctccagggcaaaagtctggggatgatcttcgaaaagaggagtactcggaccagactgtcaacagagactggattcgctctgctgggaggacacccatgctttctgaccacacaggacattcatctgggcgtgaacgagtcactgaccgacacagcccgggtgctgagcagcatggccgatgccgtgctggcacgggtctacaaacagagcgacctggataccctggctaaggaagcaagcatccccatcattaatgggctgtccgacctgtatcaccctatccagattctggccgattacctgaccctccaggagcattattctagtctgaaaggcctgacactgagctggattggggacggaaacaatatcctgcactccattatgatgtctgccgctaagtttgggatgcacctccaggcagccacaccaaaaggctacgaacccgatgccagtgtgactaagctggccgaacagtatgctaaagagaacggcactaagctgctgctgaccaatgaccccctggaggctgcacacggaggcaacgtcctgatcactgatacctggatcagcatgggccaggaggaagagaagaagaagcggctccaggccttccagggctaccaggtgacaatgaaaactgccaaggtcgccgcttctgattggacttttctgcattgtctgccccgaaaacctgaagaggtggacgatgaggtcttctattcacctaggagcctggtgtttccagaagccgagaatcgcaagtggacaatcatggccgtgatggtgtccctgctgactgactattccccacagctgcagaagcctaagttttgagatatcgtcgactcgctgatcagcctcgactgtgccttctagttgccagccatctgttgtttgcccctcccccgtgccttccttgaccctggaaggtgccactcccactgtcctttcctaataaaatgaggaaattgcatcgcattgtctgagtaggtgtcattctattctggggggtggggtggggcaggacagcaagggggaggattgggaagacaatagcaggcatgctggggatgcggtgggctctatggcttctgaggcggaaagaaccagctggggctcgactagactagtcctgcaggtagagcatggctacgtaaggaacccctagtgatggagttggccactccctctctgcgcgctcgctcgctcactgaggccgggcgaccaaaggtcgcccgacgcccgggctttgcccgggcggcctcagtgagcgagcgagcgcgcagagagggagtggccaa

SEQ ID NO: 25 - DNA, 2659 bp, Artificial sequence
  2hOTCenh.hAATprom.beta gint.hOTCco.BGHpa expression cassette
ttagggctgattgttgagacactggtgaactttgaacctctgtgatttccctgtttgctctgtgcctgatagctttcagtctgctaacaaatctcctttatgcagtttaacctctgtacttccaatggggaggaattggaatcagcctatgggagaagagatagctctaggattcttagggctgattgttgagacactggtgaactttgaacctctgtgatttccctgtttgctctgtgcctgatagctttcagtctgctaacaaatctcctttatgcagtttaacctctgtacttccaatggggaggaattggaatcagcctatgggagaagagatagctctaggattcagatcttgctaccagtggaacagccactaaggattctgcagtgagagcagagggccagctaagtggtactctcccagagactgtctgactcacgccaccccctccaccttggacacaggacgctgtggtttctgagccaggtacaatgactcctttcggtaagtgcagtggaagctgtacactgcccaggcaaagcgtccgggcagcgtaggcgggcgactcagatcccagccagtggacttagcccctgtttgctcctccgataactggggtgaccttggttaatattcaccagcagcctcccccgttgcccctctggatccactgcttaaatacggacgaggacagggccctgtctcctcagcttcaggcaccaccactgacctgggacagtgaatgcggccgctgagaacttcagggtgagtctatgggacccttgatgttttctttccccttcttttctatggttaagttcatgtcataggaaggggagaagtaacagggtacacatattgaccaaatcagggtaattttgcatttgtaattttaaaaaatgctttcttcttttaatatacttttttgtttatcttatttctaatactttccctaatctctttctttcagggcaataatgatacaatgtatcatgcctctttgcaccattctaaagaataacagtgataatttctgggttaaggcaatagcaatatttctgcatataaatatttctgcatataaattgtaactgatgtaagaggtttcatattgctaatagcagctacaatccagctaccattctgcttttattttatggttgggataaggctggattattctgagtccaagctaggcccttttgctaatcatgttcatacctcttatcttcctcccacagctcctgggcaacgtgctggtctgtgtgctggcccatcactttggcaaagcacgtgagatctgaattcgccgccaccatgctgtttaacctgagaatcctgctgaataacgctgcctttaggaacggacataacttcatggtccgcaactttcgctgtggccagcctctccagaacaaagtgcagctgaaggggagggacctgctgaccctgaaaaatttcacaggagaggaaatcaagtacatgctgtggctgtctgccgatctgaagttccggatcaagcagaagggcgaatatctgccactgctccagggcaaaagtctggggatgatcttcgaaaagaggagtactcggaccagactgtcaacagagactggattcgctctgctgggaggacacccatgctttctgaccacacaggacattcatctgggcgtgaacgagtcactgaccgacacagcccgggtgctgagcagcatggccgatgccgtgctggcacgggtctacaaacagagcgacctggataccctggctaaggaagcaagcatccccatcattaatgggctgtccgacctgtatcaccctatccagattctggccgattacctgaccctccaggagcattattctagtctgaaaggcctgacactgagctggattggggacggaaacaatatcctgcactccattatgatgtctgccgctaagtttgggatgcacctccaggcagccacaccaaaaggctacgaacccgatgccagtgtgactaagctggccgaacagtatgctaaagagaacggcactaagctgctgctgaccaatgaccccctggaggctgcacacggaggcaacgtcctgatcactgatacctggatcagcatgggccaggaggaagagaagaagaagcggctccaggccttccagggctaccaggtgacaatgaaaactgccaaggtcgccgcttctgattggacttttctgcattgtctgccccgaaaacctgaagaggtggacgatgaggtcttctattcacctaggagcctggtgtttccagaagccgagaatcgcaagtggacaatcatggccgtgatggtgtccctgctgactgactattccccacagctgcagaagcctaagttttgagatatcgtcgactcgctgatcagcctcgactgtgccttctagttgccagccatctgttgtttgcccctcccccgtgccttccttgaccctggaaggtgccactcccactgtcctttcctaataaaatgaggaaattgcatcgcattgtctgagtaggtgtcattctattctggggggtggggtggggcaggacagcaagggggaggattgggaagacaatagcaggcatgctggggatgcggtgggctctatggcttctgaggcggaaagaac

SEQ ID NO: 26 - DNA, 3037 bp, Artificial sequence
  AAV2-2hOTCenh.hAATprom.beta gint.hOTCco.BGHpa expression cassette
ttggccactccctctctgcgcgctcgctcgctcactgaggccgcccgggcaaagcccgggcgtcgggcgacctttggtcgcccggcctcagtgagcgagcgagcgcgcagagagggagtggccaactccatcactaggggttccttacgtagccatgctctagcgatcgcggtaccttaattaattagggctgattgttgagacactggtgaactttgaacctctgtgatttccctgtttgctctgtgcctgatagctttcagtctgctaacaaatctcctttatgcagtttaacctctgtacttccaatggggaggaattggaatcagcctatgggagaagagatagctctaggattcttagggctgattgttgagacactggtgaactttgaacctctgtgatttccctgtttgctctgtgcctgatagctttcagtctgctaacaaatctcctttatgcagtttaacctctgtacttccaatggggaggaattggaatcagcctatgggagaagagatagctctaggattcagatcttgctaccagtggaacagccactaaggattctgcagtgagagcagagggccagctaagtggtactctcccagagactgtctgactcacgccaccccctccaccttggacacaggacgctgtggtttctgagccaggtacaatgactcctttcggtaagtgcagtggaagctgtacactgcccaggcaaagcgtccgggcagcgtaggcgggcgactcagatcccagccagtggacttagcccctgtttgctcctccgataactggggtgaccttggttaatattcaccagcagcctcccccgttgcccctctggatccactgcttaaatacggacgaggacagggccctgtctcctcagcttcaggcaccaccactgacctgggacagtgaatgcggccgctgagaacttcagggtgagtctatgggacccttgatgttttctttccccttcttttctatggttaagttcatgtcataggaaggggagaagtaacagggtacacatattgaccaaatcagggtaattttgcatttgtaattttaaaaaatgctttcttcttttaatatacttttttgtttatcttatttctaatactttccctaatctctttctttcagggcaataatgatacaatgtatcatgcctctttgcaccattctaaagaataacagtgataatttctgggttaaggcaatagcaatatttctgcatataaatatttctgcatataaattgtaactgatgtaagaggtttcatattgctaatagcagctacaatccagctaccattctgcttttattttatggttgggataaggctggattattctgagtccaagctaggcccttttgctaatcatgttcatacctcttatcttcctcccacagctcctgggcaacgtgctggtctgtgtgctggcccatcactttggcaaagcacgtgagatctgaattcgccgccaccatgctgtttaacctgagaatcctgctgaataacgctgcctttaggaacggacataacttcatggtccgcaactttcgctgtggccagcctctccagaacaaagtgcagctgaaggggagggacctgctgaccctgaaaaatttcacaggagaggaaatcaagtacatgctgtggctgtctgccgatctgaagttccggatcaagcagaagggcgaatatctgccactgctccagggcaaaagtctggggatgatcttcgaaaagaggagtactcggaccagactgtcaacagagactggattcgctctgctgggaggacacccatgctttctgaccacacaggacattcatctgggcgtgaacgagtcactgaccgacacagcccgggtgctgagcagcatggccgatgccgtgctggcacgggtctacaaacagagcgacctggataccctggctaaggaagcaagcatccccatcattaatgggctgtccgacctgtatcaccctatccagattctggccgattacctgaccctccaggagcattattctagtctgaaaggcctgacactgagctggattggggacggaaacaatatcctgcactccattatgatgtctgccgctaagtttgggatgcacctccaggcagccacaccaaaaggctacgaacccgatgccagtgtgactaagctggccgaacagtatgctaaagagaacggcactaagctgctgctgaccaatgaccccctggaggctgcacacggaggcaacgtcctgatcactgatacctggatcagcatgggccaggaggaagagaagaagaagcggctccaggccttccagggctaccaggtgacaatgaaaactgccaaggtcgccgcttctgattggacttttctgcattgtctgccccgaaaacctgaagaggtggacgatgaggtcttctattcacctaggagcctggtgtttccagaagccgagaatcgcaagtggacaatcatggccgtgatggtgtccctgctgactgactattccccacagctgcagaagcctaagttttgagatatcgtcgactcgctgatcagcctcgactgtgccttctagttgccagccatctgttgtttgcccctcccccgtgccttccttgaccctggaaggtgccactcccactgtcctttcctaataaaatgaggaaattgcatcgcattgtctgagtaggtgtcattctattctggggggtggggtggggcaggacagcaagggggaggattgggaagacaatagcaggcatgctggggatgcggtgggctctatggcttctgaggcggaaagaaccagctggggctcgactagactagtcctgcaggtagagcatggctacgtaaggaacccctagtgatggagttggccactccctctctgcgcgctcgctcgctcactgaggccgggcgaccaaaggtcgcccgacgcccgggctttgcccgggcggcctcagtgagcgagcgagcgcgcagagagggagtggccaa

SEQ ID NO: 27 - DNA, 7338 bp, Artificial sequence
  pAAV2-hOTCenh.hOTCprom.SV40int.hOTCco.BGHpa
gctagcgatgaccctgctgattggttcgctgaccatttccgggtgcgggacggcgttaccagaaactcagaaggttcgtccaaccaaaccgactctgacggcagtttacgagagagatgatagggtctgcttcagtaagccagatgctacacaattaggcttgtacatattgtcgttagaacgcggctacaattaatacataaccttatgtatcatacacatacgatttaggtgacactatagaatacacggaattaattcttggccactccctctctgcgcgctcgctcgctcactgaggccgcccgggcaaagcccgggcgtcgggcgacctttggtcgcccggcctcagtgagcgagcgagcgcgcagagagggagtggccaactccatcactaggggttccttacgtagccatgctctagcgatcgcggtaccttaattaattagggctgattgttgagacactggtgaactttgaacctctgtgatttccctgtttgctctgtgcctgatagctttcagtctgctaacaaatctcctttatgcagtttaacctctgtacttccaatggggaggaattggaatcagcctatgggagaagagatagctctaggattcagatctacaagaaagttaaaattgaattagaggaatcatggggtcaacaagagcccctggatgaattctgaggatgaacatcaaagcctgtaaagtaaaacagactccacatgtgacataatcagcagaagctgggtagttgaaatctacccctcaacaagttcattgagatgccctgccttttgagattcagtgaaattgcttttaacttcatcccacttgtgatgcagctccccttttccaatccctctgggagttattggtatcttaacttttttttagttccctctggctttgagctcctgcatctgtagcattaggagggtttgtgagttgctttggcatctcagaaatgctgcctgtactctctagcatggaactgcagacacttcttgatttctccccaagcattaccaatatgagttgtgtgtatggctagcacagttcagtgaagatatggggtcaagctatgggctttatattagcctgtggtttggcctcatctccctcaggctccatgcaaacgttcaatttcactcctgtattatgtggagcgcttttgctctctgaaacctattcaataactggccttgtttgcctcttcaaagatgctttattatgttttttaaattcactctctcccttctcacctctgtacctttgcaagcagttgcttctgcctggaatatcctttccagaatggaagatttggtagaggttgggaaatgtcagtctttcccctcactttatctcacatcattctctgtaagtagaaggaaatggtgacaatatttatttctctactagtattaattatgacatcacaaacatctcggctcctgaggtggccatagttggtctttaaataacactttttggtattccacaaacttctggaaaatatttacttgggtttgctaaagtcatataaattgaccagaagaggcagccctacccctgcccctcctctccttcctcctacccttcctaccttagagggctcccgcttcttcgaagccagacaactttgtctggacctctcctatgggcttgtattatggatatttgtttataaatcataccacctttactgaactgtgaactctgcaaagatgatgtcatcttccctctctgaaacttcagtgcagctcggtatctgatacagaattgactttgaatcacctgatttctaactgaggataaatgaataaatgtgaagttgcagatggccccttagtgatctgaataggctgctaggggaagagcatatggtatccccacttcccacttgtactgactgtcaggtgctgttagaatcaataggcaactatttcttttctttttctttctttctttcttttttttgagacagtgtctctctctgtcacccaggctggagtacagtggtgcaatctgggctcactgcaacctctgtctcccgggttcaagcgactctcatgcctcagcctcccaaatagctgggattacaggtgtgcaccaccacgtctagctaatttttgtatttttagtggagacggggattcaccatgttggccaggctggtctcgaactcctgggctcaagtgatccgcccgcctcagcctcccaaagtgctgggattacaggcgtgagccaccgtgcccggccagcaattatttctttattgaagacttatgtgcaaggcacaaagggagctccaggactgagatatttttactataccttctctatcatcttgcacccccaaaatagcttccagggcacttctttctatttgtttttgtggaaagactggcaattagaggtagaaaagtgaaataaatggaaatagtactactcaggactgtcacatctacatctgtgtttttgcagtgccaatttgcattttctgagtgagttacttctactcaccttcacagcagccggtaccgcagtgccttgcatatattatatcctcaatgagtacttgtcaattgattttgtacatgcgtgtgacagtataaatatattatgaaaaatgaggaggccaggcaataaaagagtcaggatttcttccaaaaaaaatacacagcggtggagcttggcataaagttcaaatgctcctacaccctgccctgcagtatctctaaccaggggactttgataaggaagctgaagggtgatattacctttgctccctcactgcaactgaacacatttcttagtttttaggtggcccccgctggctaacttgctgtggcggccgctctaaggtaaatataaaatttttaagtgtataatgtgttaaactactgattctaattgtttctctcttttagattccaacctttggaactgatctagagaattcgccgccaccatgctgtttaacctgagaatcctgctgaataacgctgcctttaggaacggacataacttcatggtccgcaactttcgctgtggccagcctctccagaacaaagtgcagctgaaggggagggacctgctgaccctgaaaaatttcacaggagaggaaatcaagtacatgctgtggctgtctgccgatctgaagttccggatcaagcagaagggcgaatatctgccactgctccagggcaaaagtctggggatgatcttcgaaaagaggagtactcggaccagactgtcaacagagactggattcgctctgctgggaggacacccatgctttctgaccacacaggacattcatctgggcgtgaacgagtcactgaccgacacagcccgggtgctgagcagcatggccgatgccgtgctggcacgggtctacaaacagagcgacctggataccctggctaaggaagcaagcatccccatcattaatgggctgtccgacctgtatcaccctatccagattctggccgattacctgaccctccaggagcattattctagtctgaaaggcctgacactgagctggattggggacggaaacaatatcctgcactccattatgatgtctgccgctaagtttgggatgcacctccaggcagccacaccaaaaggctacgaacccgatgccagtgtgactaagctggccgaacagtatgctaaagagaacggcactaagctgctgctgaccaatgaccccctggaggctgcacacggaggcaacgtcctgatcactgatacctggatcagcatgggccaggaggaagagaagaagaagcggctccaggccttccagggctaccaggtgacaatgaaaactgccaaggtcgccgcttctgattggacttttctgcattgtctgccccgaaaacctgaagaggtggacgatgaggtcttctattcacctaggagcctggtgtttccagaagccgagaatcgcaagtggacaatcatggccgtgatggtgtccctgctgactgactattccccacagctgcagaagcctaagttttgagatatcgtcgactcgctgatcagcctcgactgtgccttctagttgccagccatctgttgtttgcccctcccccgtgccttccttgaccctggaaggtgccactcccactgtcctttcctaataaaatgaggaaattgcatcgcattgtctgagtaggtgtcattctattctggggggtggggtggggcaggacagcaagggggaggattgggaagacaatagcaggcatgctggggatgcggtgggctctatggcttctgaggcggaaagaaccagctggggctcgactagactagtcctgcaggtagagcatggctacgtaaggaacccctagtgatggagttggccactccctctctgcgcgctcgctcgctcactgaggccgggcgaccaaaggtcgcccgacgcccgggctttgcccgggcggcctcagtgagcgagcgagcgcgcagagagggagtggccaactttttgcaaaagcctaggcctccaaaaaagcctcctcactacttctggaatagctcagaggccgaggcggcctcggcctctgcataaataaaaaaaattagtcagccatggggcggagaatgggcggaactgggcggagttaggggcgggatgggcggagttaggggcgggactatggttgctgactaattgagatgcatgctttgcatacttctgcctgctggggagcctggggactttccacacctggttgctgactaattgagatgcatgctttgcatacttctgcctgctggggagcctggggactttccacaccctaactgacacacattccacagctgcattaatgaatcggccaacgcgcggggagaggcggtttgcgtattgggcgctcttccgcttcctcgctcactgactcgctgcgctcggtcgttcggctgcggcgagcggtatcagctcactcaaaggcggtaatacggttatccacagaatcaggggataacgcaggaaagaacatgtgagcaaaaggccagcaaaaggccaggaaccgtaaaaaggccgcgttgctggcgtttttccataggctccgcccccctgacgagcatcacaaaaatcgacgctcaagtcagaggtggcgaaacccgacaggactataaagataccaggcgtttccccctggaagctccctcgtgcgctctcctgttccgaccctgccgcttaccggatacctgtccgcctttctcccttcgggaagcgtggcgctttctcatagctcacgctgtaggtatctcagttcggtgtaggtcgttcgctccaagctgggctgtgtgcacgaaccccccgttcagcccgaccgctgcgccttatccggtaactatcgtcttgagtccaacccggtaagacacgacttatcgccactggcagcagccactggtaacaggattagcagagcgaggtatgtaggcggtgctacagagttcttgaagtggtggcctaactacggctacactagaagaacagtatttggtatctgcgctctgctgaagccagttaccttcggaaaaagagttggtagctcttgatccggcaaacaaaccaccgctggtagcggtggtttttttgtttgcaagcagcagattacgcgcagaaaaaaaggatctcaagaagatcctttgatcttttctacggggtctgacgctcagtggaacgaaaactcacgttaagggattttggtcatgagattatcaaaaaggatcttcacctagatccttttaaattaaaaatgaagttttaaatcaagcccaatctgaataatgttacaaccaattaaccaattctgattagaaaaactcatcgagcatcaaatgaaactgcaatttattcatatcaggattatcaataccatatttttgaaaaagccgtttctgtaatgaaggagaaaactcaccgaggcagttccataggatggcaagatcctggtatcggtctgcgattccgactcgtccaacatcaatacaacctattaatttcccctcgtcaaaaataaggttatcaagtgagaaatcaccatgagtgacgactgaatccggtgagaatggcaaaagtttatgcatttctttccagacttgttcaacaggccagccattacgctcgtcatcaaaatcactcgcatcaaccaaaccgttattcattcgtgattgcgcctgagcgagacgaaatacgcgatcgctgttaaaaggacaattacaaacaggaatcgaatgcaaccggcgcaggaacactgccagcgcatcaacaatattttcacctgaatcaggatattcttctaatacctggaatgctgtttttccggggatcgcagtggtgagtaaccatgcatcatcaggagtacggataaaatgcttgatggtcggaagaggcataaattccgtcagccagtttagtctgaccatctcatctgtaacatcattggcaacgctacctttgccatgtttcagaaacaactctggcgcatcgggcttcccatacaagcgatagattgtcgcacctgattgcccgacattatcgcgagcccatttatacccatataaatcagcatccatgttggaatttaatcgcggcctcgacgtttcccgttgaatatggctcataccggtactcttcctttttcaatattattgaagcatttatcagggttattgtctcatgagcggatacatatttgaatgtatttagaaaaataaacaaataggggttccgcgcacatttccccgaaaagtgccacctgacgtctaagaaaccattattatcatgacattaacctataaaaataggcgtatcacgaggccctttcgtctcgcgcgtttcggtgatgacggtgaaaacctctgacacatgcagctcccggagacggtcacagcttgtctgtaagcggatgccgggagcagacaagcccgtcagggcgcgtcagcgggtgttggcgggtgtcggggctggcttaactatgcggcatcagagcagattgtactgagagtgcaccattcgacgctctcccttatgcgactcctgcattaggaagcagcccagtagtaggttgaggccgttgagcaccgccgccgcaaggaatggtgcatgcaaggagatggcgcccaacagtcccccggccacggggcctgccaccatacccacgccgaaacaagcgctcatgagcccgaagtggcgagcccgatcttccccatcggtgatgtcggcgatataggcgccagcaaccgcacctgtggcgccggtgatgccggccacgatgcgtccggcgtagaggatctg

SEQ ID NO: 28 - DNA, 7338 bp, Artificial sequence
  pAAV2-hOTCenh.hAATprom.SV40int.hOTCco.BGHpa
gctagcgatgaccctgctgattggttcgctgaccatttccgggtgcgggacggcgttaccagaaactcagaaggttcgtccaaccaaaccgactctgacggcagtttacgagagagatgatagggtctgcttcagtaagccagatgctacacaattaggcttgtacatattgtcgttagaacgcggctacaattaatacataaccttatgtatcatacacatacgatttaggtgacactatagaatacacggaattaattcttggccactccctctctgcgcgctcgctcgctcactgaggccgcccgggcaaagcccgggcgtcgggcgacctttggtcgcccggcctcagtgagcgagcgagcgcgcagagagggagtggccaactccatcactaggggttccttacgtagccatgctctagcgatcgcggtaccttaattaattagggctgattgttgagacactggtgaactttgaacctctgtgatttccctgtttgctctgtgcctgatagctttcagtctgctaacaaatctcctttatgcagtttaacctctgtacttccaatggggaggaattggaatcagcctatgggagaagagatagctctaggattcagatctcccagtcttgtgtctgccgggcaatgagcaaggctccttcctgtccaagctccccgcccctccccagcctactgcctccacccgaagtctacttcctgggtgggcaggaactgggcactgtgcccagggcatgcactgcctccacgcagcaaccctcagagtcctgagctgaaccaagaaggaggagggggtcgggcctccgaggaaggcctagccgctgctgctgccaggaattccaggttggaggggcggcaacctcctgccagccttcaggccactctcctgtgcctgccagaagagacagagcttgaggagagcttgaggagagcaggaaaggtgggacattgctgctgctgctcactcagttccacaggtgggagggacagcagggcttagagtgggggtcattgtgcagatgggaaaacaaaggcccagagaggggaagaaatgcccaggagctaccgagggcaggcgacctcaaccacagcccagtgctggagctgtgagtggatgtagagcagcggaatatccattcagccagctcaggggaaggacaggggccctgaagccaggggatggagctgcagggaagggagctcagagagaaggggaggggagtctgagctcagtttcccgctgcctgaaaggagggtggtacctactcccttcacagggtaactgaatgagagactgcctggaggaaagctcttcaagtgtggcccaccccaccccagtgacaccagcccctgacacgggggagggagggcagcatcaggaggggctttctgggcacacccagtacccgtctctgagctttccttgaactgttgcattttaatcctcacagcagctcaacaaggtacataccgtcaccatccccattttacagatagggaaattgaggctcggagcggttaaacaactcacctgaggcctcacagccagtaagtgggttccctggtctgaatgtgtgtgctggaggatcctgtgggtcactcgcctggtagagccccaaggtggaggcataaatgggactggtgaatgacagaaggggcaaaaatgcactcatccattcactctgcaagtatctacggcacgtacgccagctcccaagcaggtttgcgggttgcacagcgggcgatgcaatctgatttaggcttttaaagggattgcaatcaagtggggccccactagcctcaaccctgtacctcccctcccctccacccccagcagtctccaaaggcctccaacaaccccagagtgggggccatgtatccaaagaaactccaagctgtatacggatcacactggttttccaggagcaaaaacagaaacaggcctgaggctggtcaaaattgaacctcctcctgctctgagcagcctggggggcagactaagcagagggctgtgcagacccacataaagagcctactgtgtgccaggcacttcacccgaggcacttcacaagcatgcttgggaatgaaacttccaactctttgggatgcaggtgaaacagttcctggttcagagaggtgaagcggcctgcctgaggcagcacagctcttctttacagatgtgcttccccacctctaccctgtctcacggccccccatgccagcctgacggttgtgtctgcctcagtcatgctccatttttccatcgggaccatcaagagggtgtttgtgtctaaggctgactgggtaactttggatgagcggtctctccgctctgagcctgtttcctcatctgtcaaatgggctctaacccactctgatctcccagggcggcagtaagtcttcagcatcaggcattttggggtgactcagtaaatggtagatcttgctaccagtggaacagccactaaggattctgcagtgagagcagagggccagctaagtggtactctcccagagactgtctgactcacgccaccccctccaccttggacacaggacgctgtggtttctgagccaggtacaatgactcctttcggtaagtgcagtggaagctgtacactgcccaggcaaagcgtccgggcagcgtaggcgggcgactcagatcccagccagtggacttagcccctgtttgctcctccgataactggggtgaccttggttaatattcaccagcagcctcccccgttgcccctctggatccactgcttaaatacggacgaggacagggccctgtctcctcagcttcaggcaccaccactgacctgggacagtgaatgcggccgctctaaggtaaatataaaatttttaagtgtataatgtgttaaactactgattctaattgtttctctcttttagattccaacctttggaactgatctagagaattcgccgccaccatgctgtttaacctgagaatcctgctgaataacgctgcctttaggaacggacataacttcatggtccgcaactttcgctgtggccagcctctccagaacaaagtgcagctgaaggggagggacctgctgaccctgaaaaatttcacaggagaggaaatcaagtacatgctgtggctgtctgccgatctgaagttccggatcaagcagaagggcgaatatctgccactgctccagggcaaaagtctggggatgatcttcgaaaagaggagtactcggaccagactgtcaacagagactggattcgctctgctgggaggacacccatgctttctgaccacacaggacattcatctgggcgtgaacgagtcactgaccgacacagcccgggtgctgagcagcatggccgatgccgtgctggcacgggtctacaaacagagcgacctggataccctggctaaggaagcaagcatccccatcattaatgggctgtccgacctgtatcaccctatccagattctggccgattacctgaccctccaggagcattattctagtctgaaaggcctgacactgagctggattggggacggaaacaatatcctgcactccattatgatgtctgccgctaagtttgggatgcacctccaggcagccacaccaaaaggctacgaacccgatgccagtgtgactaagctggccgaacagtatgctaaagagaacggcactaagctgctgctgaccaatgaccccctggaggctgcacacggaggcaacgtcctgatcactgatacctggatcagcatgggccaggaggaagagaagaagaagcggctccaggccttccagggctaccaggtgacaatgaaaactgccaaggtcgccgcttctgattggacttttctgcattgtctgccccgaaaacctgaagaggtggacgatgaggtcttctattcacctaggagcctggtgtttccagaagccgagaatcgcaagtggacaatcatggccgtgatggtgtccctgctgactgactattccccacagctgcagaagcctaagttttgagatatcgtcgactcgctgatcagcctcgactgtgccttctagttgccagccatctgttgtttgcccctcccccgtgccttccttgaccctggaaggtgccactcccactgtcctttcctaataaaatgaggaaattgcatcgcattgtctgagtaggtgtcattctattctggggggtggggtggggcaggacagcaagggggaggattgggaagacaatagcaggcatgctggggatgcggtgggctctatggcttctgaggcggaaagaaccagctggggctcgactagactagtcctgcaggtagagcatggctacgtaaggaacccctagtgatggagttggccactccctctctgcgcgctcgctcgctcactgaggccgggcgaccaaaggtcgcccgacgcccgggctttgcccgggcggcctcagtgagcgagcgagcgcgcagagagggagtggccaactttttgcaaaagcctaggcctccaaaaaagcctcctcactacttctggaatagctcagaggccgaggcggcctcggcctctgcataaataaaaaaaattagtcagccatggggcggagaatgggcggaactgggcggagttaggggcgggatgggcggagttaggggcgggactatggttgctgactaattgagatgcatgctttgcatacttctgcctgctggggagcctggggactttccacacctggttgctgactaattgagatgcatgctttgcatacttctgcctgctggggagcctggggactttccacaccctaactgacacacattccacagctgcattaatgaatcggccaacgcgcggggagaggcggtttgcgtattgggcgctcttccgcttcctcgctcactgactcgctgcgctcggtcgttcggctgcggcgagcggtatcagctcactcaaaggcggtaatacggttatccacagaatcaggggataacgcaggaaagaacatgtgagcaaaaggccagcaaaaggccaggaaccgtaaaaaggccgcgttgctggcgtttttccataggctccgcccccctgacgagcatcacaaaaatcgacgctcaagtcagaggtggcgaaacccgacaggactataaagataccaggcgtttccccctggaagctccctcgtgcgctctcctgttccgaccctgccgcttaccggatacctgtccgcctttctcccttcgggaagcgtggcgctttctcatagctcacgctgtaggtatctcagttcggtgtaggtcgttcgctccaagctgggctgtgtgcacgaaccccccgttcagcccgaccgctgcgccttatccggtaactatcgtcttgagtccaacccggtaagacacgacttatcgccactggcagcagccactggtaacaggattagcagagcgaggtatgtaggcggtgctacagagttcttgaagtggtggcctaactacggctacactagaagaacagtatttggtatctgcgctctgctgaagccagttaccttcggaaaaagagttggtagctcttgatccggcaaacaaaccaccgctggtagcggtggtttttttgtttgcaagcagcagattacgcgcagaaaaaaaggatctcaagaagatcctttgatcttttctacggggtctgacgctcagtggaacgaaaactcacgttaagggattttggtcatgagattatcaaaaaggatcttcacctagatccttttaaattaaaaatgaagttttaaatcaagcccaatctgaataatgttacaaccaattaaccaattctgattagaaaaactcatcgagcatcaaatgaaactgcaatttattcatatcaggattatcaataccatatttttgaaaaagccgtttctgtaatgaaggagaaaactcaccgaggcagttccataggatggcaagatcctggtatcggtctgcgattccgactcgtccaacatcaatacaacctattaatttcccctcgtcaaaaataaggttatcaagtgagaaatcaccatgagtgacgactgaatccggtgagaatggcaaaagtttatgcatttctttccagacttgttcaacaggccagccattacgctcgtcatcaaaatcactcgcatcaaccaaaccgttattcattcgtgattgcgcctgagcgagacgaaatacgcgatcgctgttaaaaggacaattacaaacaggaatcgaatgcaaccggcgcaggaacactgccagcgcatcaacaatattttcacctgaatcaggatattcttctaatacctggaatgctgtttttccggggatcgcagtggtgagtaaccatgcatcatcaggagtacggataaaatgcttgatggtcggaagaggcataaattccgtcagccagtttagtctgaccatctcatctgtaacatcattggcaacgctacctttgccatgtttcagaaacaactctggcgcatcgggcttcccatacaagcgatagattgtcgcacctgattgcccgacattatcgcgagcccatttatacccatataaatcagcatccatgttggaatttaatcgcggcctcgacgtttcccgttgaatatggctcataccggtactcttcctttttcaatattattgaagcatttatcagggttattgtctcatgagcggatacatatttgaatgtatttagaaaaataaacaaataggggttccgcgcacatttccccgaaaagtgccacctgacgtctaagaaaccattattatcatgacattaacctataaaaataggcgtatcacgaggccctttcgtctcgcgcgtttcggtgatgacggtgaaaacctctgacacatgcagctcccggagacggtcacagcttgtctgtaagcggatgccgggagcagacaagcccgtcagggcgcgtcagcgggtgttggcgggtgtcggggctggcttaactatgcggcatcagagcagattgtactgagagtgcaccattcgacgctctcccttatgcgactcctgcattaggaagcagcccagtagtaggttgaggccgttgagcaccgccgccgcaaggaatggtgcatgcaaggagatggcgcccaacagtcccccggccacggggcctgccaccatacccacgccgaaacaagcgctcatgagcccgaagtggcgagcccgatcttccccatcggtgatgtcggcgatataggcgccagcaaccgcacctgtggcgccggtgatgccggccacgatgcgtccggcgtagaggatctg

SEQ ID NO: 29 - DNA, 6108 bp, Artificial sequence
  pAAV2-2hOTCenh.hOTCprom.SV40int.hOTCco.BGHpa
gctagcgatgaccctgctgattggttcgctgaccatttccgggtgcgggacggcgttaccagaaactcagaaggttcgtccaaccaaaccgactctgacggcagtttacgagagagatgatagggtctgcttcagtaagccagatgctacacaattaggcttgtacatattgtcgttagaacgcggctacaattaatacataaccttatgtatcatacacatacgatttaggtgacactatagaatacacggaattaattcttggccactccctctctgcgcgctcgctcgctcactgaggccgcccgggcaaagcccgggcgtcgggcgacctttggtcgcccggcctcagtgagcgagcgagcgcgcagagagggagtggccaactccatcactaggggttccttacgtagccatgctctagcgatcgcggtaccttaattaattagggctgattgttgagacactggtgaactttgaacctctgtgatttccctgtttgctctgtgcctgatagctttcagtctgctaacaaatctcctttatgcagtttaacctctgtacttccaatggggaggaattggaatcagcctatgggagaagagatagctctaggattcttagggctgattgttgagacactggtgaactttgaacctctgtgatttccctgtttgctctgtgcctgatagctttcagtctgctaacaaatctcctttatgcagtttaacctctgtacttccaatggggaggaattggaatcagcctatgggagaagagatagctctaggattcagatctcaagcgactctcatgcctcagcctcccaaatagctgggattacaggtgtgcaccaccacgtctagctaatttttgtatttttagtggagacggggattcatcatgttggccaggctggtctcgaactcctgggctcaagtgatccgcccgcctcagcctcccaaagtgctgggattataggcgtgagccaccatgcccggccagcaattatttctttattgaagacttatgtgcaaggcacaaagggagctccaggactgagatatttttactataccttctctatcatcttgcacccccaaaatagcttccagggcacttctatttgtttttgtggaaagactggcaattagaggtagaaaagtgaaataaatggaaatagtactactcagggctgtcacatctacatctgtgtttttgcagtgccaatttgcattttctgagtgagttacttctactcaccttcacagcagccagtaccgcagtgccttgcatatattatatcctcaatgagtacttgtcaattgattttgtacatgcgtgtgacagtataaatatattatgaaaaatgaggaggccaggcaataaaagagtcaggatttcttccaaaaaaaatacacagcggtggagcttggcataaagttcaaatgctcctacaccctgccctgcagtatctctaaccaggggactttgataaggaagctgaagggtgatattacctttgctccctcactgcaactgaacacatttcttagtttttaggtggcccccgctggctaacttgctgtggcggccgctctaaggtaaatataaaatttttaagtgtataatgtgttaaactactgattctaattgtttctctcttttagattccaacctttggaactgatctagagaattcgccgccaccatgctgtttaacctgagaatcctgctgaataacgctgcctttaggaacggacataacttcatggtccgcaactttcgctgtggccagcctctccagaacaaagtgcagctgaaggggagggacctgctgaccctgaaaaatttcacaggagaggaaatcaagtacatgctgtggctgtctgccgatctgaagttccggatcaagcagaagggcgaatatctgccactgctccagggcaaaagtctggggatgatcttcgaaaagaggagtactcggaccagactgtcaacagagactggattcgctctgctgggaggacacccatgctttctgaccacacaggacattcatctgggcgtgaacgagtcactgaccgacacagcccgggtgctgagcagcatggccgatgccgtgctggcacgggtctacaaacagagcgacctggataccctggctaaggaagcaagcatccccatcattaatgggctgtccgacctgtatcaccctatccagattctggccgattacctgaccctccaggagcattattctagtctgaaaggcctgacactgagctggattggggacggaaacaatatcctgcactccattatgatgtctgccgctaagtttgggatgcacctccaggcagccacaccaaaaggctacgaacccgatgccagtgtgactaagctggccgaacagtatgctaaagagaacggcactaagctgctgctgaccaatgaccccctggaggctgcacacggaggcaacgtcctgatcactgatacctggatcagcatgggccaggaggaagagaagaagaagcggctccaggccttccagggctaccaggtgacaatgaaaactgccaaggtcgccgcttctgattggacttttctgcattgtctgccccgaaaacctgaagaggtggacgatgaggtcttctattcacctaggagcctggtgtttccagaagccgagaatcgcaagtggacaatcatggccgtgatggtgtccctgctgactgactattccccacagctgcagaagcctaagttttgagatatcgtcgactcgctgatcagcctcgactgtgccttctagttgccagccatctgttgtttgcccctcccccgtgccttccttgaccctggaaggtgccactcccactgtcctttcctaataaaatgaggaaattgcatcgcattgtctgagtaggtgtcattctattctggggggtggggtggggcaggacagcaagggggaggattgggaagacaatagcaggcatgctggggatgcggtgggctctatggcttctgaggcggaaagaaccagctggggctcgactagactagtcctgcaggtagagcatggctacgtaaggaacccctagtgatggagttggccactccctctctgcgcgctcgctcgctcactgaggccgggcgaccaaaggtcgcccgacgcccgggctttgcccgggcggcctcagtgagcgagcgagcgcgcagagagggagtggccaactttttgcaaaagcctaggcctccaaaaaagcctcctcactacttctggaatagctcagaggccgaggcggcctcggcctctgcataaataaaaaaaattagtcagccatggggcggagaatgggcggaactgggcggagttaggggcgggatgggcggagttaggggcgggactatggttgctgactaattgagatgcatgctttgcatacttctgcctgctggggagcctggggactttccacacctggttgctgactaattgagatgcatgctttgcatacttctgcctgctggggagcctggggactttccacaccctaactgacacacattccacagctgcattaatgaatcggccaacgcgcggggagaggcggtttgcgtattgggcgctcttccgcttcctcgctcactgactcgctgcgctcggtcgttcggctgcggcgagcggtatcagctcactcaaaggcggtaatacggttatccacagaatcaggggataacgcaggaaagaacatgtgagcaaaaggccagcaaaaggccaggaaccgtaaaaaggccgcgttgctggcgtttttccataggctccgcccccctgacgagcatcacaaaaatcgacgctcaagtcagaggtggcgaaacccgacaggactataaagataccaggcgtttccccctggaagctccctcgtgcgctctcctgttccgaccctgccgcttaccggatacctgtccgcctttctcccttcgggaagcgtggcgctttctcatagctcacgctgtaggtatctcagttcggtgtaggtcgttcgctccaagctgggctgtgtgcacgaaccccccgttcagcccgaccgctgcgccttatccggtaactatcgtcttgagtccaacccggtaagacacgacttatcgccactggcagcagccactggtaacaggattagcagagcgaggtatgtaggcggtgctacagagttcttgaagtggtggcctaactacggctacactagaagaacagtatttggtatctgcgctctgctgaagccagttaccttcggaaaaagagttggtagctcttgatccggcaaacaaaccaccgctggtagcggtggtttttttgtttgcaagcagcagattacgcgcagaaaaaaaggatctcaagaagatcctttgatcttttctacggggtctgacgctcagtggaacgaaaactcacgttaagggattttggtcatgagattatcaaaaaggatcttcacctagatccttttaaattaaaaatgaagttttaaatcaatctaaagtatatatgagtaaacttggtctgacagttaccaatgcttaatcagtgaggcacctatctcagcgatctgtctatttcgttcatccatagttgcctgactccccgtcgtgtagataactacgatacgggagggcttaccatctggccccagtgctgcaatgataccgcgagacccacgctcaccggctccagatttatcagcaataaaccagccagccggaagggccgagcgcagaagtggtcctgcaactttatccgcctccatccagtctattaattgttgccgggaagctagagtaagtagttcgccagttaatagtttgcgcaacgttgttgccattgctacaggcatcgtggtgtcacgctcgtcgtttggtatggcttcattcagctccggttcccaacgatcaaggcgagttacatgatcccccatgttgtgcaaaaaagcggttagctccttcggtcctccgatcgttgtcagaagtaagttggccgcagtgttatcactcatggttatggcagcactgcataattctcttactgtcatgccatccgtaagatgcttttctgtgactggtgagtactcaaccaagtcattctgagaatagtgtatgcggcgaccgagttgctcttgcccggcgtcaatacgggataataccgcgccacatagcagaactttaaaagtgctcatcattggaaaacgttcttcggggcgaaaactctcaaggatcttaccgctgttgagatccagttcgatgtaacccactcgtgcacccaactgatcttcagcatcttttactttcaccagcgtttctgggtgagcaaaaacaggaaggcaaaatgccgcaaaaaagggaataagggcgacacggaaatgttgaatactcatactcttcctttttcaatattattgaagcatttatcagggttattgtctcatgagcggatacatatttgaatgtatttagaaaaataaacaaataggggttccgcgcacatttccccgaaaagtgccacctgacgtctaagaaaccattattatcatgacattaacctataaaaataggcgtatcacgaggccctttcgtctcgcgcgtttcggtgatgacggtgaaaacctctgacacatgcagctcccggagacggtcacagcttgtctgtaagcggatgccgggagcagacaagcccgtcagggcgcgtcagcgggtgttggcgggtgtcggggctggcttaactatgcggcatcagagcagattgtactgagagtgcaccattcgacgctctcccttatgcgactcctgcattaggaagcagcccagtagtaggttgaggccgttgagcaccgccgccgcaaggaatggtgcatgcaaggagatggcgcccaacagtcccccggccacggggcctgccaccatacccacgccgaaacaagcgctcatgagcccgaagtggcgagcccgatcttccccatcggtgatgtcggcgatataggcgccagcaaccgcacctgtggcgccggtgatgccggccacgatgcgtccggcgtagaggatctg

SEQ ID NO: 30 - DNA, 6554 bp, Artificial sequence
  pAAV2-2hOTCenh.hOTCprom.beta gint.hOTCco.BGHpa
gctagcgatgaccctgctgattggttcgctgaccatttccgggtgcgggacggcgttaccagaaactcagaaggttcgtccaaccaaaccgactctgacggcagtttacgagagagatgatagggtctgcttcagtaagccagatgctacacaattaggcttgtacatattgtcgttagaacgcggctacaattaatacataaccttatgtatcatacacatacgatttaggtgacactatagaatacacggaattaattcttggccactccctctctgcgcgctcgctcgctcactgaggccgcccgggcaaagcccgggcgtcgggcgacctttggtcgcccggcctcagtgagcgagcgagcgcgcagagagggagtggccaactccatcactaggggttccttacgtagccatgctctagcgatcgcggtaccttaattaattagggctgattgttgagacactggtgaactttgaacctctgtgatttccctgtttgctctgtgcctgatagctttcagtctgctaacaaatctcctttatgcagtttaacctctgtacttccaatggggaggaattggaatcagcctatgggagaagagatagctctaggattcttagggctgattgttgagacactggtgaactttgaacctctgtgatttccctgtttgctctgtgcctgatagctttcagtctgctaacaaatctcctttatgcagtttaacctctgtacttccaatggggaggaattggaatcagcctatgggagaagagatagctctaggattcagatctcaagcgactctcatgcctcagcctcccaaatagctgggattacaggtgtgcaccaccacgtctagctaatttttgtatttttagtggagacggggattcatcatgttggccaggctggtctcgaactcctgggctcaagtgatccgcccgcctcagcctcccaaagtgctgggattataggcgtgagccaccatgcccggccagcaattatttctttattgaagacttatgtgcaaggcacaaagggagctccaggactgagatatttttactataccttctctatcatcttgcacccccaaaatagcttccagggcacttctatttgtttttgtggaaagactggcaattagaggtagaaaagtgaaataaatggaaatagtactactcagggctgtcacatctacatctgtgtttttgcagtgccaatttgcattttctgagtgagttacttctactcaccttcacagcagccagtaccgcagtgccttgcatatattatatcctcaatgagtacttgtcaattgattttgtacatgcgtgtgacagtataaatatattatgaaaaatgaggaggccaggcaataaaagagtcaggatttcttccaaaaaaaatacacagcggtggagcttggcataaagttcaaatgctcctacaccctgccctgcagtatctctaaccaggggactttgataaggaagctgaagggtgatattacctttgctccctcactgcaactgaacacatttcttagtttttaggtggcccccgctggctaacttgctgtggcggccgctgagaacttcagggtgagtctatgggacccttgatgttttctttccccttcttttctatggttaagttcatgtcataggaaggggagaagtaacagggtacacatattgaccaaatcagggtaattttgcatttgtaattttaaaaaatgctttcttcttttaatatacttttttgtttatcttatttctaatactttccctaatctctttctttcagggcaataatgatacaatgtatcatgcctctttgcaccattctaaagaataacagtgataatttctgggttaaggcaatagcaatatttctgcatataaatatttctgcatataaattgtaactgatgtaagaggtttcatattgctaatagcagctacaatccagctaccattctgcttttattttatggttgggataaggctggattattctgagtccaagctaggcccttttgctaatcatgttcatacctcttatcttcctcccacagctcctgggcaacgtgctggtctgtgtgctggcccatcactttggcaaagcacgtggaattcgccgccaccatgctgtttaacctgagaatcctgctgaataacgctgcctttaggaacggacataacttcatggtccgcaactttcgctgtggccagcctctccagaacaaagtgcagctgaaggggagggacctgctgaccctgaaaaatttcacaggagaggaaatcaagtacatgctgtggctgtctgccgatctgaagttccggatcaagcagaagggcgaatatctgccactgctccagggcaaaagtctggggatgatcttcgaaaagaggagtactcggaccagactgtcaacagagactggattcgctctgctgggaggacacccatgctttctgaccacacaggacattcatctgggcgtgaacgagtcactgaccgacacagcccgggtgctgagcagcatggccgatgccgtgctggcacgggtctacaaacagagcgacctggataccctggctaaggaagcaagcatccccatcattaatgggctgtccgacctgtatcaccctatccagattctggccgattacctgaccctccaggagcattattctagtctgaaaggcctgacactgagctggattggggacggaaacaatatcctgcactccattatgatgtctgccgctaagtttgggatgcacctccaggcagccacaccaaaaggctacgaacccgatgccagtgtgactaagctggccgaacagtatgctaaagagaacggcactaagctgctgctgaccaatgaccccctggaggctgcacacggaggcaacgtcctgatcactgatacctggatcagcatgggccaggaggaagagaagaagaagcggctccaggccttccagggctaccaggtgacaatgaaaactgccaaggtcgccgcttctgattggacttttctgcattgtctgccccgaaaacctgaagaggtggacgatgaggtcttctattcacctaggagcctggtgtttccagaagccgagaatcgcaagtggacaatcatggccgtgatggtgtccctgctgactgactattccccacagctgcagaagcctaagttttgagatatcgtcgactcgctgatcagcctcgactgtgccttctagttgccagccatctgttgtttgcccctcccccgtgccttccttgaccctggaaggtgccactcccactgtcctttcctaataaaatgaggaaattgcatcgcattgtctgagtaggtgtcattctattctggggggtggggtggggcaggacagcaagggggaggattgggaagacaatagcaggcatgctggggatgcggtgggctctatggcttctgaggcggaaagaaccagctggggctcgactagactagtcctgcaggtagagcatggctacgtaaggaacccctagtgatggagttggccactccctctctgcgcgctcgctcgctcactgaggccgggcgaccaaaggtcgcccgacgcccgggctttgcccgggcggcctcagtgagcgagcgagcgcgcagagagggagtggccaactttttgcaaaagcctaggcctccaaaaaagcctcctcactacttctggaatagctcagaggccgaggcggcctcggcctctgcataaataaaaaaaattagtcagccatggggcggagaatgggcggaactgggcggagttaggggcgggatgggcggagttaggggcgggactatggttgctgactaattgagatgcatgctttgcatacttctgcctgctggggagcctggggactttccacacctggttgctgactaattgagatgcatgctttgcatacttctgcctgctggggagcctggggactttccacaccctaactgacacacattccacagctgcattaatgaatcggccaacgcgcggggagaggcggtttgcgtattgggcgctcttccgcttcctcgctcactgactcgctgcgctcggtcgttcggctgcggcgagcggtatcagctcactcaaaggcggtaatacggttatccacagaatcaggggataacgcaggaaagaacatgtgagcaaaaggccagcaaaaggccaggaaccgtaaaaaggccgcgttgctggcgtttttccataggctccgcccccctgacgagcatcacaaaaatcgacgctcaagtcagaggtggcgaaacccgacaggactataaagataccaggcgtttccccctggaagctccctcgtgcgctctcctgttccgaccctgccgcttaccggatacctgtccgcctttctcccttcgggaagcgtggcgctttctcatagctcacgctgtaggtatctcagttcggtgtaggtcgttcgctccaagctgggctgtgtgcacgaaccccccgttcagcccgaccgctgcgccttatccggtaactatcgtcttgagtccaacccggtaagacacgacttatcgccactggcagcagccactggtaacaggattagcagagcgaggtatgtaggcggtgctacagagttcttgaagtggtggcctaactacggctacactagaagaacagtatttggtatctgcgctctgctgaagccagttaccttcggaaaaagagttggtagctcttgatccggcaaacaaaccaccgctggtagcggtggtttttttgtttgcaagcagcagattacgcgcagaaaaaaaggatctcaagaagatcctttgatcttttctacggggtctgacgctcagtggaacgaaaactcacgttaagggattttggtcatgagattatcaaaaaggatcttcacctagatccttttaaattaaaaatgaagttttaaatcaatctaaagtatatatgagtaaacttggtctgacagttaccaatgcttaatcagtgaggcacctatctcagcgatctgtctatttcgttcatccatagttgcctgactccccgtcgtgtagataactacgatacgggagggcttaccatctggccccagtgctgcaatgataccgcgagacccacgctcaccggctccagatttatcagcaataaaccagccagccggaagggccgagcgcagaagtggtcctgcaactttatccgcctccatccagtctattaattgttgccgggaagctagagtaagtagttcgccagttaatagtttgcgcaacgttgttgccattgctacaggcatcgtggtgtcacgctcgtcgtttggtatggcttcattcagctccggttcccaacgatcaaggcgagttacatgatcccccatgttgtgcaaaaaagcggttagctccttcggtcctccgatcgttgtcagaagtaagttggccgcagtgttatcactcatggttatggcagcactgcataattctcttactgtcatgccatccgtaagatgcttttctgtgactggtgagtactcaaccaagtcattctgagaatagtgtatgcggcgaccgagttgctcttgcccggcgtcaatacgggataataccgcgccacatagcagaactttaaaagtgctcatcattggaaaacgttcttcggggcgaaaactctcaaggatcttaccgctgttgagatccagttcgatgtaacccactcgtgcacccaactgatcttcagcatcttttactttcaccagcgtttctgggtgagcaaaaacaggaaggcaaaatgccgcaaaaaagggaataagggcgacacggaaatgttgaatactcatactcttcctttttcaatattattgaagcatttatcagggttattgtctcatgagcggatacatatttgaatgtatttagaaaaataaacaaataggggttccgcgcacatttccccgaaaagtgccacctgacgtctaagaaaccattattatcatgacattaacctataaaaataggcgtatcacgaggccctttcgtctcgcgcgtttcggtgatgacggtgaaaacctctgacacatgcagctcccggagacggtcacagcttgtctgtaagcggatgccgggagcagacaagcccgtcagggcgcgtcagcgggtgttggcgggtgtcggggctggcttaactatgcggcatcagagcagattgtactgagagtgcaccattcgacgctctcccttatgcgactcctgcattaggaagcagcccagtagtaggttgaggccgttgagcaccgccgccgcaaggaatggtgcatgcaaggagatggcgcccaacagtcccccggccacggggcctgccaccatacccacgccgaaacaagcgctcatgagcccgaagtggcgagcccgatcttccccatcggtgatgtcggcgatataggcgccagcaaccgcacctgtggcgccggtgatgccggccacgatgcgtccggcgtagaggatctg

SEQ ID NO: 31 - DNA, 5711 bp, Artificial sequence
  pAAV2-2hOTCenh.hAATprom.SV40int.hOTCco.BGHpa
gctagcgatgaccctgctgattggttcgctgaccatttccgggtgcgggacggcgttaccagaaactcagaaggttcgtccaaccaaaccgactctgacggcagtttacgagagagatgatagggtctgcttcagtaagccagatgctacacaattaggcttgtacatattgtcgttagaacgcggctacaattaatacataaccttatgtatcatacacatacgatttaggtgacactatagaatacacggaattaattcttggccactccctctctgcgcgctcgctcgctcactgaggccgcccgggcaaagcccgggcgtcgggcgacctttggtcgcccggcctcagtgagcgagcgagcgcgcagagagggagtggccaactccatcactaggggttccttacgtagccatgctctagcgatcgcggtaccttaattaattagggctgattgttgagacactggtgaactttgaacctctgtgatttccctgtttgctctgtgcctgatagctttcagtctgctaacaaatctcctttatgcagtttaacctctgtacttccaatggggaggaattggaatcagcctatgggagaagagatagctctaggattcttagggctgattgttgagacactggtgaactttgaacctctgtgatttccctgtttgctctgtgcctgatagctttcagtctgctaacaaatctcctttatgcagtttaacctctgtacttccaatggggaggaattggaatcagcctatgggagaagagatagctctaggattcagatcttgctaccagtggaacagccactaaggattctgcagtgagagcagagggccagctaagtggtactctcccagagactgtctgactcacgccaccccctccaccttggacacaggacgctgtggtttctgagccaggtacaatgactcctttcggtaagtgcagtggaagctgtacactgcccaggcaaagcgtccgggcagcgtaggcgggcgactcagatcccagccagtggacttagcccctgtttgctcctccgataactggggtgaccttggttaatattcaccagcagcctcccccgttgcccctctggatccactgcttaaatacggacgaggacagggccctgtctcctcagcttcaggcaccaccactgacctgggacagtgaatgcggccgctctaaggtaaatataaaatttttaagtgtataatgtgttaaactactgattctaattgtttctctcttttagattccaacctttggaactgatctagagaattcgccgccaccatgctgtttaacctgagaatcctgctgaataacgctgcctttaggaacggacataacttcatggtccgcaactttcgctgtggccagcctctccagaacaaagtgcagctgaaggggagggacctgctgaccctgaaaaatttcacaggagaggaaatcaagtacatgctgtggctgtctgccgatctgaagttccggatcaagcagaagggcgaatatctgccactgctccagggcaaaagtctggggatgatcttcgaaaagaggagtactcggaccagactgtcaacagagactggattcgctctgctgggaggacacccatgctttctgaccacacaggacattcatctgggcgtgaacgagtcactgaccgacacagcccgggtgctgagcagcatggccgatgccgtgctggcacgggtctacaaacagagcgacctggataccctggctaaggaagcaagcatccccatcattaatgggctgtccgacctgtatcaccctatccagattctggccgattacctgaccctccaggagcattattctagtctgaaaggcctgacactgagctggattggggacggaaacaatatcctgcactccattatgatgtctgccgctaagtttgggatgcacctccaggcagccacaccaaaaggctacgaacccgatgccagtgtgactaagctggccgaacagtatgctaaagagaacggcactaagctgctgctgaccaatgaccccctggaggctgcacacggaggcaacgtcctgatcactgatacctggatcagcatgggccaggaggaagagaagaagaagcggctccaggccttccagggctaccaggtgacaatgaaaactgccaaggtcgccgcttctgattggacttttctgcattgtctgccccgaaaacctgaagaggtggacgatgaggtcttctattcacctaggagcctggtgtttccagaagccgagaatcgcaagtggacaatcatggccgtgatggtgtccctgctgactgactattccccacagctgcagaagcctaagttttgagatatcgtcgactcgctgatcagcctcgactgtgccttctagttgccagccatctgttgtttgcccctcccccgtgccttccttgaccctggaaggtgccactcccactgtcctttcctaataaaatgaggaaattgcatcgcattgtctgagtaggtgtcattctattctggggggtggggtggggcaggacagcaagggggaggattgggaagacaatagcaggcatgctggggatgcggtgggctctatggcttctgaggcggaaagaaccagctggggctcgactagactagtcctgcaggtagagcatggctacgtaaggaacccctagtgatggagttggccactccctctctgcgcgctcgctcgctcactgaggccgggcgaccaaaggtcgcccgacgcccgggctttgcccgggcggcctcagtgagcgagcgagcgcgcagagagggagtggccaactttttgcaaaagcctaggcctccaaaaaagcctcctcactacttctggaatagctcagaggccgaggcggcctcggcctctgcataaataaaaaaaattagtcagccatggggcggagaatgggcggaactgggcggagttaggggcgggatgggcggagttaggggcgggactatggttgctgactaattgagatgcatgctttgcatacttctgcctgctggggagcctggggactttccacacctggttgctgactaattgagatgcatgctttgcatacttctgcctgctggggagcctggggactttccacaccctaactgacacacattccacagctgcattaatgaatcggccaacgcgcggggagaggcggtttgcgtattgggcgctcttccgcttcctcgctcactgactcgctgcgctcggtcgttcggctgcggcgagcggtatcagctcactcaaaggcggtaatacggttatccacagaatcaggggataacgcaggaaagaacatgtgagcaaaaggccagcaaaaggccaggaaccgtaaaaaggccgcgttgctggcgtttttccataggctccgcccccctgacgagcatcacaaaaatcgacgctcaagtcagaggtggcgaaacccgacaggactataaagataccaggcgtttccccctggaagctccctcgtgcgctctcctgttccgaccctgccgcttaccggatacctgtccgcctttctcccttcgggaagcgtggcgctttctcatagctcacgctgtaggtatctcagttcggtgtaggtcgttcgctccaagctgggctgtgtgcacgaaccccccgttcagcccgaccgctgcgccttatccggtaactatcgtcttgagtccaacccggtaagacacgacttatcgccactggcagcagccactggtaacaggattagcagagcgaggtatgtaggcggtgctacagagttcttgaagtggtggcctaactacggctacactagaagaacagtatttggtatctgcgctctgctgaagccagttaccttcggaaaaagagttggtagctcttgatccggcaaacaaaccaccgctggtagcggtggtttttttgtttgcaagcagcagattacgcgcagaaaaaaaggatctcaagaagatcctttgatcttttctacggggtctgacgctcagtggaacgaaaactcacgttaagggattttggtcatgagattatcaaaaaggatcttcacctagatccttttaaattaaaaatgaagttttaaatcaatctaaagtatatatgagtaaacttggtctgacagttaccaatgcttaatcagtgaggcacctatctcagcgatctgtctatttcgttcatccatagttgcctgactccccgtcgtgtagataactacgatacgggagggcttaccatctggccccagtgctgcaatgataccgcgagacccacgctcaccggctccagatttatcagcaataaaccagccagccggaagggccgagcgcagaagtggtcctgcaactttatccgcctccatccagtctattaattgttgccgggaagctagagtaagtagttcgccagttaatagtttgcgcaacgttgttgccattgctacaggcatcgtggtgtcacgctcgtcgtttggtatggcttcattcagctccggttcccaacgatcaaggcgagttacatgatcccccatgttgtgcaaaaaagcggttagctccttcggtcctccgatcgttgtcagaagtaagttggccgcagtgttatcactcatggttatggcagcactgcataattctcttactgtcatgccatccgtaagatgcttttctgtgactggtgagtactcaaccaagtcattctgagaatagtgtatgcggcgaccgagttgctcttgcccggcgtcaatacgggataataccgcgccacatagcagaactttaaaagtgctcatcattggaaaacgttcttcggggcgaaaactctcaaggatcttaccgctgttgagatccagttcgatgtaacccactcgtgcacccaactgatcttcagcatcttttactttcaccagcgtttctgggtgagcaaaaacaggaaggcaaaatgccgcaaaaaagggaataagggcgacacggaaatgttgaatactcatactcttcctttttcaatattattgaagcatttatcagggttattgtctcatgagcggatacatatttgaatgtatttagaaaaataaacaaataggggttccgcgcacatttccccgaaaagtgccacctgacgtctaagaaaccattattatcatgacattaacctataaaaataggcgtatcacgaggccctttcgtctcgcgcgtttcggtgatgacggtgaaaacctctgacacatgcagctcccggagacggtcacagcttgtctgtaagcggatgccgggagcagacaagcccgtcagggcgcgtcagcgggtgttggcgggtgtcggggctggcttaactatgcggcatcagagcagattgtactgagagtgcaccattcgacgctctcccttatgcgactcctgcattaggaagcagcccagtagtaggttgaggccgttgagcaccgccgccgcaaggaatggtgcatgcaaggagatggcgcccaacagtcccccggccacggggcctgccaccatacccacgccgaaacaagcgctcatgagcccgaagtggcgagcccgatcttccccatcggtgatgtcggcgatataggcgccagcaaccgcacctgtggcgccggtgatgccggccacgatgcgtccggcgtagaggatctg

SEQ ID NO: 32 - DNA, 6163 bp, Artificial sequence
  pAAV2-2hOTCenh.hAATprom.beta gint.hOTCco.BGHpa
gctagcgatgaccctgctgattggttcgctgaccatttccgggtgcgggacggcgttaccagaaactcagaaggttcgtccaaccaaaccgactctgacggcagtttacgagagagatgatagggtctgcttcagtaagccagatgctacacaattaggcttgtacatattgtcgttagaacgcggctacaattaatacataaccttatgtatcatacacatacgatttaggtgacactatagaatacacggaattaattcttggccactccctctctgcgcgctcgctcgctcactgaggccgcccgggcaaagcccgggcgtcgggcgacctttggtcgcccggcctcagtgagcgagcgagcgcgcagagagggagtggccaactccatcactaggggttccttacgtagccatgctctagcgatcgcggtaccttaattaattagggctgattgttgagacactggtgaactttgaacctctgtgatttccctgtttgctctgtgcctgatagctttcagtctgctaacaaatctcctttatgcagtttaacctctgtacttccaatggggaggaattggaatcagcctatgggagaagagatagctctaggattcttagggctgattgttgagacactggtgaactttgaacctctgtgatttccctgtttgctctgtgcctgatagctttcagtctgctaacaaatctcctttatgcagtttaacctctgtacttccaatggggaggaattggaatcagcctatgggagaagagatagctctaggattcagatcttgctaccagtggaacagccactaaggattctgcagtgagagcagagggccagctaagtggtactctcccagagactgtctgactcacgccaccccctccaccttggacacaggacgctgtggtttctgagccaggtacaatgactcctttcggtaagtgcagtggaagctgtacactgcccaggcaaagcgtccgggcagcgtaggcgggcgactcagatcccagccagtggacttagcccctgtttgctcctccgataactggggtgaccttggttaatattcaccagcagcctcccccgttgcccctctggatccactgcttaaatacggacgaggacagggccctgtctcctcagcttcaggcaccaccactgacctgggacagtgaatgcggccgctgagaacttcagggtgagtctatgggacccttgatgttttctttccccttcttttctatggttaagttcatgtcataggaaggggagaagtaacagggtacacatattgaccaaatcagggtaattttgcatttgtaattttaaaaaatgctttcttcttttaatatacttttttgtttatcttatttctaatactttccctaatctctttctttcagggcaataatgatacaatgtatcatgcctctttgcaccattctaaagaataacagtgataatttctgggttaaggcaatagcaatatttctgcatataaatatttctgcatataaattgtaactgatgtaagaggtttcatattgctaatagcagctacaatccagctaccattctgcttttattttatggttgggataaggctggattattctgagtccaagctaggcccttttgctaatcatgttcatacctcttatcttcctcccacagctcctgggcaacgtgctggtctgtgtgctggcccatcactttggcaaagcacgtgagatctgaattcgccgccaccatgctgtttaacctgagaatcctgctgaataacgctgcctttaggaacggacataacttcatggtccgcaactttcgctgtggccagcctctccagaacaaagtgcagctgaaggggagggacctgctgaccctgaaaaatttcacaggagaggaaatcaagtacatgctgtggctgtctgccgatctgaagttccggatcaagcagaagggcgaatatctgccactgctccagggcaaaagtctggggatgatcttcgaaaagaggagtactcggaccagactgtcaacagagactggattcgctctgctgggaggacacccatgctttctgaccacacaggacattcatctgggcgtgaacgagtcactgaccgacacagcccgggtgctgagcagcatggccgatgccgtgctggcacgggtctacaaacagagcgacctggataccctggctaaggaagcaagcatccccatcattaatgggctgtccgacctgtatcaccctatccagattctggccgattacctgaccctccaggagcattattctagtctgaaaggcctgacactgagctggattggggacggaaacaatatcctgcactccattatgatgtctgccgctaagtttgggatgcacctccaggcagccacaccaaaaggctacgaacccgatgccagtgtgactaagctggccgaacagtatgctaaagagaacggcactaagctgctgctgaccaatgaccccctggaggctgcacacggaggcaacgtcctgatcactgatacctggatcagcatgggccaggaggaagagaagaagaagcggctccaggccttccagggctaccaggtgacaatgaaaactgccaaggtcgccgcttctgattggacttttctgcattgtctgccccgaaaacctgaagaggtggacgatgaggtcttctattcacctaggagcctggtgtttccagaagccgagaatcgcaagtggacaatcatggccgtgatggtgtccctgctgactgactattccccacagctgcagaagcctaagttttgagatatcgtcgactcgctgatcagcctcgactgtgccttctagttgccagccatctgttgtttgcccctcccccgtgccttccttgaccctggaaggtgccactcccactgtcctttcctaataaaatgaggaaattgcatcgcattgtctgagtaggtgtcattctattctggggggtggggtggggcaggacagcaagggggaggattgggaagacaatagcaggcatgctggggatgcggtgggctctatggcttctgaggcggaaagaaccagctggggctcgactagactagtcctgcaggtagagcatggctacgtaaggaacccctagtgatggagttggccactccctctctgcgcgctcgctcgctcactgaggccgggcgaccaaaggtcgcccgacgcccgggctttgcccgggcggcctcagtgagcgagcgagcgcgcagagagggagtggccaactttttgcaaaagcctaggcctccaaaaaagcctcctcactacttctggaatagctcagaggccgaggcggcctcggcctctgcataaataaaaaaaattagtcagccatggggcggagaatgggcggaactgggcggagttaggggcgggatgggcggagttaggggcgggactatggttgctgactaattgagatgcatgctttgcatacttctgcctgctggggagcctggggactttccacacctggttgctgactaattgagatgcatgctttgcatacttctgcctgctggggagcctggggactttccacaccctaactgacacacattccacagctgcattaatgaatcggccaacgcgcggggagaggcggtttgcgtattgggcgctcttccgcttcctcgctcactgactcgctgcgctcggtcgttcggctgcggcgagcggtatcagctcactcaaaggcggtaatacggttatccacagaatcaggggataacgcaggaaagaacatgtgagcaaaaggccagcaaaaggccaggaaccgtaaaaaggccgcgttgctggcgtttttccataggctccgcccccctgacgagcatcacaaaaatcgacgctcaagtcagaggtggcgaaacccgacaggactataaagataccaggcgtttccccctggaagctccctcgtgcgctctcctgttccgaccctgccgcttaccggatacctgtccgcctttctcccttcgggaagcgtggcgctttctcatagctcacgctgtaggtatctcagttcggtgtaggtcgttcgctccaagctgggctgtgtgcacgaaccccccgttcagcccgaccgctgcgccttatccggtaactatcgtcttgagtccaacccggtaagacacgacttatcgccactggcagcagccactggtaacaggattagcagagcgaggtatgtaggcggtgctacagagttcttgaagtggtggcctaactacggctacactagaagaacagtatttggtatctgcgctctgctgaagccagttaccttcggaaaaagagttggtagctcttgatccggcaaacaaaccaccgctggtagcggtggtttttttgtttgcaagcagcagattacgcgcagaaaaaaaggatctcaagaagatcctttgatcttttctacggggtctgacgctcagtggaacgaaaactcacgttaagggattttggtcatgagattatcaaaaaggatcttcacctagatccttttaaattaaaaatgaagttttaaatcaatctaaagtatatatgagtaaacttggtctgacagttaccaatgcttaatcagtgaggcacctatctcagcgatctgtctatttcgttcatccatagttgcctgactccccgtcgtgtagataactacgatacgggagggcttaccatctggccccagtgctgcaatgataccgcgagacccacgctcaccggctccagatttatcagcaataaaccagccagccggaagggccgagcgcagaagtggtcctgcaactttatccgcctccatccagtctattaattgttgccgggaagctagagtaagtagttcgccagttaatagtttgcgcaacgttgttgccattgctacaggcatcgtggtgtcacgctcgtcgtttggtatggcttcattcagctccggttcccaacgatcaaggcgagttacatgatcccccatgttgtgcaaaaaagcggttagctccttcggtcctccgatcgttgtcagaagtaagttggccgcagtgttatcactcatggttatggcagcactgcataattctcttactgtcatgccatccgtaagatgcttttctgtgactggtgagtactcaaccaagtcattctgagaatagtgtatgcggcgaccgagttgctcttgcccggcgtcaatacgggataataccgcgccacatagcagaactttaaaagtgctcatcattggaaaacgttcttcggggcgaaaactctcaaggatcttaccgctgttgagatccagttcgatgtaacccactcgtgcacccaactgatcttcagcatcttttactttcaccagcgtttctgggtgagcaaaaacaggaaggcaaaatgccgcaaaaaagggaataagggcgacacggaaatgttgaatactcatactcttcctttttcaatattattgaagcatttatcagggttattgtctcatgagcggatacatatttgaatgtatttagaaaaataaacaaataggggttccgcgcacatttccccgaaaagtgccacctgacgtctaagaaaccattattatcatgacattaacctataaaaataggcgtatcacgaggccctttcgtctcgcgcgtttcggtgatgacggtgaaaacctctgacacatgcagctcccggagacggtcacagcttgtctgtaagcggatgccgggagcagacaagcccgtcagggcgcgtcagcgggtgttggcgggtgtcggggctggcttaactatgcggcatcagagcagattgtactgagagtgcaccattcgacgctctcccttatgcgactcctgcattaggaagcagcccagtagtaggttgaggccgttgagcaccgccgccgcaaggaatggtgcatgcaaggagatggcgcccaacagtcccccggccacggggcctgccaccatacccacgccgaaacaagcgctcatgagcccgaagtggcgagcccgatcttccccatcggtgatgtcggcgatataggcgccagcaaccgcacctgtggcgccggtgatgccggccacgatgcgtccggcgtagaggatctg

SEQ ID NO: 33 - DNA, 20 bp, Artificial sequence
  OTC forward primer
cgatgccagtgtgactaagc

SEQ ID NO: 34 - DNA, 20 bp, Artificial sequence
  OTC reverse primer
ggagccgcttcttcttctct

SEQ ID NO: 35 - DNA, 19 bp, Artificial sequence
  GAPDH forward primer
acggcaaattcaacggcac

SEQ ID NO: 36 - DNA, 20 bp, Artificial sequence
  GAPDH reverse primer
tagtggggtctcgctcctgg